European Patent Specification EP 4 376 874 B1, published March 4, 2026. Title: CHIMERIC TIM4 RECEPTORS AND USES THEREOF. Applicant: CERO THERAPEUTICS, INC. Application WO. The sequence listing filed with the application follows.

SEQUENCE LISTING (349 sequences)

SEQ ID NO: 1 - protein, 378 aa, Homo sapiens
MSKEPLILWLMIEFWWLYLTPVTSETVVTEVLGHRVTLPCLYSSWSHNSNSMCWGKDQCPYSGCKEALIRTDGMRVTSRKSAKYRLQGTIPRGDVSLTILNPSESDSGVYCCRIEVPGWFNDVKINVRLNLQRASTTTHRTATTTTRRTTTTSPTTTRQMTTTPAALPTTVVTTPDLTTGTPLQMTTIAVFTTANTCLSLTPSTLPEEATGLLTPEPSKEGPILTAESETVLPSDSWSSVESTSADTVLLTSKESKVWDLPSTSHVSMWKTSDSVSSPQPGASDTAVPEQNKTTKTGQMDGIPMSMKNEMPISQLLMIIAPSLGFVLFALFVAFLLRGKLMETYCSQKHTRLDYIGDSKNVLNDVQHGREDEDGLFTL

SEQ ID NO: 2 - protein, 279 aa, Mus musculus
MSKGLLLLWLVTELWWLYLTPAASEDTIIGFLGQPVTLPCHYLSWSQSRNSMCWGKGSCPNSKCNAELLRTDGTRIISRKSTKYTLLGKVQFGEVSLTISNTNRGDSGVYCCRIEVPGWFNDVKKNVRLELRRATTTKKPTTTTRPTTTPYVTTTTPELLPTTVMTTSVLPTTTPPQTLATTAFSTAVTTCPSTTPGSFSQETTKGSAFTTESETLPASNHSQRSMMTISTDIAVLRPTGSNPGILPSTSQLTTQKTTLTTSESLQKTTKSHQINSRQT

SEQ ID NO: 3 - protein, 111 aa, Homo sapiens
ETVVTEVLGHRVTLPCLYSSWSHNSNSMCWGKDQCPYSGCKEALIRTDGMRVTSRKSAKYRLQGTIPRGDVSLTILNPSESDSGVYCCRIEVPGWFNDVKINVRLNLQRAS

SEQ ID NO: 4 - protein, 179 aa, Homo sapiens
TTTHRTATTTTRRTTTTSPTTTRQMTTTPAALPTTVVTTPDLTTGTPLQMTTIAVFTTANTCLSLTPSTLPEEATGLLTPEPSKEGPILTAESETVLPSDSWSSVESTSADTVLLTSKESKVWDLPSTSHVSMWKTSDSVSSPQPGASDTAVPEQNKTTKTGQMDGIPMSMKNEMPISQ

SEQ ID NO: 5 - protein, 314 aa, Homo sapiens
MSKEPLILWLMIEFWWLYLTPVTSETVVTEVLGHRVTLPCLYSSWSHNSNSMCWGKDQCPYSGCKEALIRTDGMRVTSRKSAKYRLQGTIPRGDVSLTILNPSESDSGVYCCRIEVPGWFNDVKINVRLNLQRASTTTHRTATTTTRRTTTTSPTTTRQMTTTPAALPTTVVTTPDLTTGTPLQMTTIAVFTTANTCLSLTPSTLPEEATGLLTPEPSKEGPILTAESETVLPSDSWSSVESTSADTVLLTSKESKVWDLPSTSHVSMWKTSDSVSSPQPGASDTAVPEQNKTTKTGQMDGIPMSMKNEMPISQ

SEQ ID NO: 6 - protein, 290 aa, Homo sapiens [sequence omitted]

SEQ ID NO: 7 - protein, 24 aa, Homo sapiens
MSKEPLILWLMIEFWWLYLTPVTS

SEQ ID NO: 8 - protein, 22 aa, Mus musculus
MSKGLLLLWLVTELWWLYLTPA

SEQ ID NO: 9 - protein, 12 aa, synthetic construct
ESKYGPPCPPCP

SEQ ID NO: 10 - protein, 39 aa, Homo sapiens
IEVMYPPPYLDNEKSNGTIIHVKGKHLCPSPLFPGPSKP

SEQ ID NO: 11 - protein, 27 aa, Homo sapiens
FWVLVVVGGVLACYSLLVTVAFIIFWV

SEQ ID NO: 12 - protein, 41 aa, Homo sapiens
RSKRSRLLHSDYMNMTPRRPGPTRKHYQPYAPPRDFAAYRS

SEQ ID NO: 13 - protein, 41 aa, synthetic construct
RSKRSRGGHSDYMNMTPRRPGPTRKHYQPYAPPRDFAAYRS

SEQ ID NO: 14 - protein, 113 aa, Homo sapiens
RVKFSRSADAPAYQQGQNQLYNELNLGRREEYDVLDKRRGRDPEMGGKPQRRKNPQEGLYNELQKDKMAEAYSEIGMKGERRRGKGHDGLYQGLSTATKDTYDALHMQALPPR

SEQ ID NO: 15 - protein, 112 aa, synthetic construct
RVKFSRSADAPAYQQGQNQLYNELNLGRREEYDVLDKRRGRDPEMGGKPRRKNPQEGLYNELQKDKMAEAYSEIGMKGERRRGKGHDGLYQGLSTATKDTYDALHMQALPPR

SEQ ID NO: 16 - protein, 175 aa, Homo sapiens
HRFHGLWYMKMMWAWLQAKRKPRKAPSRNICYDAFVSYSERDAYWVENLMVQELENFNPPFKLCLHKRDFIPGKWIIDNIIDSIEKSHKTVFVLSENFVKSEWCKYELDFSHFRLFDENNDAAILILLEPIEKKAIPQRFCKLRKIMNTKTYLEWPMDEAQREGFWVNLRAAIKS

SEQ ID NO: 17 - protein, 146 aa, Homo sapiens
  source 1..146: note = TLR2 TIR signaling domain
ICYDAFVSYSERDAYWVENLMVQELENFNPPFKLCLHKRDFIPGKWIIDNIIDSIEKSHKTVFVLSENFVKSEWCKYELDFSHFRLFDENNDAAILILLEPIEKKAIPQRFCKLRKIMNTKTYLEWPMDEAQREGFWVNLRAAIKS

SEQ ID NO: 18 - protein, 641 aa, synthetic construct
  source 1..641: note = CER-1234
  SIGNAL 1..24
MSKEPLILWLMIEFWWLYLTPVTSETVVTEVLGHRVTLPCLYSSWSHNSNSMCWGKDQCPYSGCKEALIRTDGMRVTSRKSAKYRLQGTIPRGDVSLTILNPSESDSGVYCCRIEVPGWFNDVKINVRLNLQRASTTTHRTATTTTRRTTTTSPTTTRQMTTTPAALPTTVVTTPDLTTGTPLQMTTIAVFTTANTCLSLTPSTLPEEATGLLTPEPSKEGPILTAESETVLPSDSWSSVESTSADTVLLTSKESKVWDLPSTSHVSMWKTSDSVSSPQPGASDTAVPEQNKTTKTGQMDGIPMSMKNEMPISQFWVLVVVGGVLACYSLLVTVAFIIFWVRSKRSRLLHSDYMNMTPRRPGPTRKHYQPYAPPRDFAAYRSICYDAFVSYSERDAYWVENLMVQELENFNPPFKLCLHKRDFIPGKWIIDNIIDSIEKSHKTVFVLSENFVKSEWCKYELDFSHFRLFDENNDAAILILLEPIEKKAIPQRFCKLRKIMNTKTYLEWPMDEAQREGFWVNLRAAIKSRVKFSRSADAPAYQQGQNQLYNELNLGRREEYDVLDKRRGRDPEMGGKPQRRKNPQEGLYNELQKDKMAEAYSEIGMKGERRRGKGHDGLYQGLSTATKDTYDALHMQALPPR

SEQ ID NO: 19 - protein, 641 aa, synthetic construct
  source 1..641: note = CER-1236 (also referred to as CER1107)
  SIGNAL 1..24
MSKEPLILWLMIEFWWLYLTPVTSETVVTEVLGHRVTLPCLYSSWSHNSNSMCWGKDQCPYSGCKEALIRTDGMRVTSRKSAKYRLQGTIPRGDVSLTILNPSESDSGVYCCRIEVPGWFNDVKINVRLNLQRASTTTHRTATTTTRRTTTTSPTTTRQMTTTPAALPTTVVTTPDLTTGTPLQMTTIAVFTTANTCLSLTPSTLPEEATGLLTPEPSKEGPILTAESETVLPSDSWSSVESTSADTVLLTSKESKVWDLPSTSHVSMWKTSDSVSSPQPGASDTAVPEQNKTTKTGQMDGIPMSMKNEMPISQFWVLVVVGGVLACYSLLVTVAFIIFWVRSKRSRLLHSDYMNMTPRRPGPTRKHYQPYAPPRDFAAYRSRVKFSRSADAPAYQQGQNQLYNELNLGRREEYDVLDKRRGRDPEMGGKPQRRKNPQEGLYNELQKDKMAEAYSEIGMKGERRRGKGHDGLYQGLSTATKDTYDALHMQALPPRICYDAFVSYSERDAYWVENLMVQELENFNPPFKLCLHKRDFIPGKWIIDNIIDSIEKSHKTVFVLSENFVKSEWCKYELDFSHFRLFDENNDAAILILLEPIEKKAIPQRFCKLRKIMNTKTYLEWPMDEAQREGFWVNLRAAIKS

SEQ ID NO: 20 - protein, 377 aa, synthetic construct
MSKEPLILWLMIEFWWLYLTPVTSETVVTEVLGHRVTLPCLYSSWSHNSNSMCWGKDQCPYSGCKEALIRTDGMRVTSRKSAKYRLQGTIPRGDVSLTILNPSESDSGVYCCRIEVPGWFNDVKINVRLNLQRASTTTHRTATTTTRRTTTTSPTTTRQMTTTPAALPTTVVTTPDLTTGTPLQMTTIAVFTTANTCLSLTPSTLPEEATGLLTPEPSKEGPILTAESETVLPSDSWSSVESTSADTVLLTSKESKVWDLPSTSHVSMWKTSDSVSSPQPGASDTAVPEQNKTTKTGQMDGIPMSMKNEMPISQLLMIIAPSLGFVLFALFVAFLRGKLMETYCSQKHTRLDYIGDSKNVLNDVQHGREDEDGLFTL

SEQ ID NO: 21 - protein, 495 aa, synthetic construct
MSKEPLILWLMIEFWWLYLTPVTSETVVTEVLGHRVTLPCLYSSWSHNSNSMCWGKDQCPYSGCKEALIRTDGMRVTSRKSAKYRLQGTIPRGDVSLTILNPSESDSGVYCCRIEVPGWFNDVKINVRLNLQRASTTTHRTATTTTRRTTTTSPTTTRQMTTTPAALPTTVVTTPDLTTGTPLQMTTIAVFTTANTCLSLTPSTLPEEATGLLTPEPSKEGPILTAESETVLPSDSWSSVESTSADTVLLTSKESKVWDLPSTSHVSMWKTSDSVSSPQPGASDTAVPEQNKTTKTGQMDGIPMSMKNEMPISQFWVLVVVGGVLACYSLLVTVAFIIFWVRSKRSRLLHSDYMNMTPRRPGPTRKHYQPYAPPRDFAAYRSRVKFSRSADAPAYQQGQNQLYNELNLGRREEYDVLDKRRGRDPEMGGKPQRRKNPQEGLYNELQKDKMAEAYSEIGMKGERRRGKGHDGLYQGLSTATKDTYDALHMQALPPR

SEQ ID NO: 22 - protein, 670 aa, synthetic construct
MSKEPLILWLMIEFWWLYLTPVTSETVVTEVLGHRVTLPCLYSSWSHNSNSMCWGKDQCPYSGCKEALIRTDGMRVTSRKSAKYRLQGTIPRGDVSLTILNPSESDSGVYCCRIEVPGWFNDVKINVRLNLQRASTTTHRTATTTTRRTTTTSPTTTRQMTTTPAALPTTVVTTPDLTTGTPLQMTTIAVFTTANTCLSLTPSTLPEEATGLLTPEPSKEGPILTAESETVLPSDSWSSVESTSADTVLLTSKESKVWDLPSTSHVSMWKTSDSVSSPQPGASDTAVPEQNKTTKTGQMDGIPMSMKNEMPISQFWVLVVVGGVLACYSLLVTVAFIIFWVRSKRSRLLHSDYMNMTPRRPGPTRKHYQPYAPPRDFAAYRSHRFHGLWYMKMMWAWLQAKRKPRKAPSRNICYDAFVSYSERDAYWVENLMVQELENFNPPFKLCLHKRDFIPGKWIIDNIIDSIEKSHKTVFVLSENFVKSEWCKYELDFSHFRLFDENNDAAILILLEPIEKKAIPQRFCKLRKIMNTKTYLEWPMDEAQREGFWVNLRAAIKSRVKFSRSADAPAYQQGQNQLYNELNLGRREEYDVLDKRRGRDPEMGGKPQRRKNPQEGLYNELQKDKMAEAYSEIGMKGERRRGKGHDGLYQGLSTATKDTYDALHMQALPPR

SEQ ID NO: 23 - protein, 670 aa, synthetic construct
MSKEPLILWLMIEFWWLYLTPVTSETVVTEVLGHRVTLPCLYSSWSHNSNSMCWGKDQCPYSGCKEALIRTDGMRVTSRKSAKYRLQGTIPRGDVSLTILNPSESDSGVYCCRIEVPGWFNDVKINVRLNLQRASTTTHRTATTTTRRTTTTSPTTTRQMTTTPAALPTTVVTTPDLTTGTPLQMTTIAVFTTANTCLSLTPSTLPEEATGLLTPEPSKEGPILTAESETVLPSDSWSSVESTSADTVLLTSKESKVWDLPSTSHVSMWKTSDSVSSPQPGASDTAVPEQNKTTKTGQMDGIPMSMKNEMPISQFWVLVVVGGVLACYSLLVTVAFIIFWVRSKRSRLLHSDYMNMTPRRPGPTRKHYQPYAPPRDFAAYRSRVKFSRSADAPAYQQGQNQLYNELNLGRREEYDVLDKRRGRDPEMGGKPQRRKNPQEGLYNELQKDKMAEAYSEIGMKGERRRGKGHDGLYQGLSTATKDTYDALHMQALPPRHRFHGLWYMKMMWAWLQAKRKPRKAPSRNICYDAFVSYSERDAYWVENLMVQELENFNPPFKLCLHKRDFIPGKWIIDNIIDSIEKSHKTVFVLSENFVKSEWCKYELDFSHFRLFDENNDAAILILLEPIEKKAIPQRFCKLRKIMNTKTYLEWPMDEAQREGFWVNLRAAIKS

SEQ ID NO: 24 - protein, 641 aa, synthetic construct
MSKEPLILWLMIEFWWLYLTPVTSETVVTEVLGHRVTLPCLYSSWSHNSNSMCWGKDQCPYSGCKEALIRTDGMRVTSRKSAKYRLQGTIPRGDVSLTILNPSESDSGVYCCRIEVPGAAAAVKINVRLNLQRASTTTHRTATTTTRRTTTTSPTTTRQMTTTPAALPTTVVTTPDLTTGTPLQMTTIAVFTTANTCLSLTPSTLPEEATGLLTPEPSKEGPILTAESETVLPSDSWSSVESTSADTVLLTSKESKVWDLPSTSHVSMWKTSDSVSSPQPGASDTAVPEQNKTTKTGQMDGIPMSMKNEMPISQFWVLVVVGGVLACYSLLVTVAFIIFWVRSKRSRLLHSDYMNMTPRRPGPTRKHYQPYAPPRDFAAYRSICYDAFVSYSERDAYWVENLMVQELENFNPPFKLCLHKRDFIPGKWIIDNIIDSIEKSHKTVFVLSENFVKSEWCKYELDFSHFRLFDENNDAAILILLEPIEKKAIPQRFCKLRKIMNTKTYLEWPMDEAQREGFWVNLRAAIKSRVKFSRSADAPAYQQGQNQLYNELNLGRREEYDVLDKRRGRDPEMGGKPQRRKNPQEGLYNELQKDKMAEAYSEIGMKGERRRGKGHDGLYQGLSTATKDTYDALHMQALPPR

SEQ ID NO: 25 - protein, 641 aa, synthetic construct
MSKEPLILWLMIEFWWLYLTPVTSETVVTEVLGHRVTLPCLYSSWSHNSNSMCWGKDQCPYSGCKEALIRTDGMRVTSRKSAKYRLQGTIPRGDVSLTILNPSESDSGVYCCRIEVPGAAAAVKINVRLNLQRASTTTHRTATTTTRRTTTTSPTTTRQMTTTPAALPTTVVTTPDLTTGTPLQMTTIAVFTTANTCLSLTPSTLPEEATGLLTPEPSKEGPILTAESETVLPSDSWSSVESTSADTVLLTSKESKVWDLPSTSHVSMWKTSDSVSSPQPGASDTAVPEQNKTTKTGQMDGIPMSMKNEMPISQFWVLVVVGGVLACYSLLVTVAFIIFWVRSKRSRLLHSDYMNMTPRRPGPTRKHYQPYAPPRDFAAYRSRVKFSRSADAPAYQQGQNQLYNELNLGRREEYDVLDKRRGRDPEMGGKPQRRKNPQEGLYNELQKDKMAEAYSEIGMKGERRRGKGHDGLYQGLSTATKDTYDALHMQALPPRICYDAFVSYSERDAYWVENLMVQELENFNPPFKLCLHKRDFIPGKWIIDNIIDSIEKSHKTVFVLSENFVKSEWCKYELDFSHFRLFDENNDAAILILLEPIEKKAIPQRFCKLRKIMNTKTYLEWPMDEAQREGFWVNLRAAIKS

SEQ ID NO: 26 - protein, 444 aa, synthetic construct
MALPVTALLLPLALLLHADIQMTQTTSSLSASLGDRVTISCRASQDISKYLNWYQQKPDGTVKLLIYHTSRLHSGVPSRFSGSGSGTDYSLTISNLEQEDIATYFCQQGNTLPYTFGGGTKLEITGSTSGSGKPGSGEGSTKGEVKLQESGPGLVAPSQSLSVTCTVSGVSLPDYGVSWIRQPPRKGLEWLGVIWGSETTYYNSALKSRLTIIKDNSKSQVFLKMNSLQTDDTAIYYCAKHYYYGGSYAMDYWGQGTSVTVSSFWVLVVVGGVLACYSLLVTVAFIIFWVRSKRSRLLHSDYMNMTPRRPGPTRKHYQPYAPPRDFAAYRSRVKFSRSADAPAYQQGQNQLYNELNLGRREEYDVLDKRRGRDPEMGGKPQRRKNPQEGLYNELQKDKMAEAYSEIGMKGERRRGKGHDGLYQGLSTATKDTYDALHMQALPPR

SEQ ID NO: 27 - protein, 22 aa, Homo sapiens
MLLLVTSLLLCELPHPAFLLIP

SEQ ID NO: 28 - protein, 20 aa, synthetic construct
MHPQVVILSLILHLADSVAG

SEQ ID NO: 29 - protein, 18 aa, synthetic construct
EGRGSLLTCGDVEENPGP

SEQ ID NO: 30 - protein, 18 aa, synthetic construct
EGRGSLLTCGDVEENPGP

SEQ ID NO: 31 - protein, 23 aa, synthetic construct
LEGGGEGRGSLLTCGDVEENPGP

SEQ ID NO: 32 - protein, 19 aa, synthetic construct
EGRGSLLTCGDVEENPGPR

SEQ ID NO: 33 - protein, 24 aa, synthetic construct
LEGGGEGRGSLLTCGDVEENPGPR

SEQ ID NO: 34 - protein, 19 aa, synthetic construct
ATNFSLLKQAGDVEENPGP

SEQ ID NO: 35 - protein, 27 aa, synthetic construct
RAKRSGSGATNFSLLKQAGDVEENPGP

SEQ ID NO: 36 - protein, 20 aa, synthetic construct
QCTNYALLKLAGDVESNPGP

SEQ ID NO: 37 - protein, 22 aa, synthetic construct
VKQTLNFDLLKLAGDVESNPGP

SEQ ID NO: 38 - protein, 285 aa, synthetic construct
RKVCNGIGIGEFKDSLSINATNIKHFKNCTSISGDLHILPVAFRGDSFTHTPPLDPQELDILKTVKEITGFLLIQAWPENRTDLHAFENLEIIRGRTKQHGQFSLAVVSLNITSLGLRSLKEISDGDVIISGNKNLCYANTINWKKLFGTSGQKTKIISNRGENSCKATGQVCHALCSPEGCWGPEPRDCVSCRNVSRGRECVDKCNLLEGEPREFVENSECIQCHPECLPQAMNITCTGRGPDNCIQCAHYIDGPHCVKTCPAGVMGENNTLVWKYADAGHVCH

SEQ ID NO: 39 - protein, 300 aa, synthetic construct
RSKRSRLLHSDYMNMTPRRPGPTRKHYQPYAPPRDFAAYRSICYDAFVSYSERDAYWVENLMVQELENFNPPFKLCLHKRDFIPGKWIIDNIIDSIEKSHKTVFVLSENFVKSEWCKYELDFSHFRLFDENNDAAILILLEPIEKKAIPQRFCKLRKIMNTKTYLEWPMDEAQREGFWVNLRAAIKSRVKFSRSADAPAYQQGQNQLYNELNLGRREEYDVLDKRRGRDPEMGGKPQRRKNPQEGLYNELQKDKMAEAYSEIGMKGERRRGKGHDGLYQGLSTATKDTYDALHMQALPPR

SEQ ID NO: 40 - protein, 300 aa, synthetic construct
RSKRSRLLHSDYMNMTPRRPGPTRKHYQPYAPPRDFAAYRSRVKFSRSADAPAYQQGQNQLYNELNLGRREEYDVLDKRRGRDPEMGGKPQRRKNPQEGLYNELQKDKMAEAYSEIGMKGERRRGKGHDGLYQGLSTATKDTYDALHMQALPPRICYDAFVSYSERDAYWVENLMVQELENFNPPFKLCLHKRDFIPGKWIIDNIIDSIEKSHKTVFVLSENFVKSEWCKYELDFSHFRLFDENNDAAILILLEPIEKKAIPQRFCKLRKIMNTKTYLEWPMDEAQREGFWVNLRAAIKS

SEQ ID NO: 41 - protein, 192 aa, Homo sapiens
MQAIKCVVVGDGAVGKTCLLISYTTNAFPGEYIPTVFDNYSANVMVDGKPVNLGLWDTAGQEDYDRLRPLSYPQTDVFLICFSLVSPASFENVRAKWYPEVRHHCPNTPIILVGTKLDLRDDKDTIEKLKEKKLTPITYPQGLAMAKEIGAVKYLECSALTQRGLKTVFDEAIRAVLCPPPVKKRKRKCLLL

SEQ ID NO: 42 - protein, 215 aa, Homo sapiens
MASRGATRPNGPNTGNKICQFKLVLLGESAVGKSSLVLRFVKGQFHEFQESTIGAAFLTQTVCLDDTTVKFEIWDTAGQERYHSLAPMYYRGAQAAIVVYDITNEESFARAKNWVKELQRQASPNIVIALSGNKADLANKRAVDFQEAQSYADDNSLLFMETSAKTSMNVNEIFMAIAKKLPKNEPQNPGANSARGRGVDLTEPTQPTRNQCCSN

SEQ ID NO: 43 - protein, 207 aa, Homo sapiens
MTSRKKVLLKVIILGDSGVGKTSLMNQYVNKKFSNQYKATIGADFLTKEVMVDDRLVTMQIWDTAGQERFQSLGVAFYRGADCCVLVFDVTAPNTFKTLDSWRDEFLIQASPRDPENFPFVVLGNKIDLENRQVATKRAQAWCYSKNNIPYFETSAKEAINVEQAFQTIARNALKQETEVELYNEFPEPIKLDKNDRAKASAESCSC

SEQ ID NO: 44 - protein, 184 aa, Homo sapiens
MREYKLVVLGSGGVGKSALTVQFVQGIFVEKYDPTIEDSYRKQVEVDCQQCMLEILDTAGTEQFTAMRDLYMKNGQGFALVYSITAQSTFNDLQDLREQILRVKDTEDVPMILVGNKCDLEDERVVGKEQGQNLARQWCNCAFLESSAKSKINVNEIFYDLVRQINRKTPVEKKKPKKKSCLLL

SEQ ID NO: 45 - protein, 193 aa, Homo sapiens
MAAIRKKLVIVGDGACGKTCLLIVFSKDQFPEVYVPTVFENYVADIEVDGKQVELALWDTAGQEDYDRLRPLSYPDTDVILMCFSIDSPDSLENIPEKWTPEVKHFCPNVPIILVGNKKDLRNDEHTRRELAKMKQEPVKPEEGRDMANRIGAFGYMECSAKTKDGVREVFEMATRAALQARRGKKKSGCLVL

SEQ ID NO: 46 - protein, 191 aa, Homo sapiens
MQTIKCVVVGDGAVGKTCLLISYTTNKFPSEYVPTVFDNYAVTVMIGGEPYTLGLFDTAGQEDYDRLRPLSYPQTDVFLVCFSVVSPSSFENVKEKWVPEITHHCPKTPFLLVGTQIDLRDDPSTIEKLAKNKQKPITPETAEKLARDLKAVKYVECSALTQKGLKNVFDEAILAALEPPEPKKSRRCVLL

SEQ ID NO: 47-100 - skipped (54 entries)

SEQ ID NO: 101 - protein, 5 aa, synthetic construct
GYLMS

SEQ ID NO: 102 - protein, 17 aa, synthetic construct
VISYDGSNKYYADSVKG

SEQ ID NO: 103 - protein, 10 aa, synthetic construct
ARRDTNLFDY

SEQ ID NO: 104 - protein, 11 aa, synthetic construct
RASQSISSYLN

SEQ ID NO: 105 - protein, 7 aa, synthetic construct
AASSLQS

SEQ ID NO: 106 - protein, 9 aa, synthetic construct
QQSYSTPPT

SEQ ID NO: 107 - protein, 5 aa, synthetic construct
SYYMH

SEQ ID NO: 108 - protein, 17 aa, synthetic construct
IINPSGGGTSYAQKFQG

SEQ ID NO: 109 - protein, 12 aa, synthetic construct
DYYVTYDSWFDS

SEQ ID NO: 110 - protein, 11 aa, synthetic construct
QGDSLRSYYAS

SEQ ID NO: 111 - protein, 7 aa, synthetic construct
GKNNRPS

SEQ ID NO: 112 - protein, 11 aa, synthetic construct
NSRDSSGNHVV

SEQ ID NO: 113 - protein, 114 aa, synthetic construct
LVESGGGLVQPGGSLRLSCAASGFTFSGYLMSWVRQAPGKGLEWVAVISYDGSNKYYADSVKGRFTISRDNSKNTLYLQMDSLRAEDTAVYYCARARRDTNLFDYWGQGTLVTV

SEQ ID NO: 114 - protein, 104 aa, synthetic construct
ELTQSPSSLSASVGDRVTITCRASQSISSYLNWYQQKPGKAPKLLIYAASSLQSGVPSRFSGSGSGTDFTLTISSLQPEDFATYYCQQSYSTPPTFGQGTKVEI

SEQ ID NO: 115 - protein, 117 aa, synthetic construct
LVQSGAEVKKPGASVKVSCKASGYTFTSYYMHWVRQAPGQGLEWMGIINPSGGGTSYAQKFQGRVTMTRDTSTSTVYMELSSLRSEDTAVYYCARDYYVTYDSWFDSWGQGTLVTVS

SEQ ID NO: 116 - protein, 98 aa, synthetic construct
VSVALGQTVRITCQGDSLRSYYASWYQQKPGQAPVLVIYGKNNRPSGIPDRFSGSSSGNTASLTITGAQAEDEADYYCNSRDSSGNHVVFGGGTKLTV

SEQ ID NO: 117 - protein, 120 aa, synthetic construct
AEVQLVESGGGVVQPGRSLRLSCAASGFTFSDYTMSWVRQAPGKGLEWVAVISYDGSNKYYADSVKGRFTISRDNSKNTLYLQMNSLRAEDTAVYYCAKDRGSAQGYPLDYWGQGTLVTV

SEQ ID NO: 118 - protein, 115 aa, synthetic construct
SELDIQMTQSPPTLSLSPGERATLSCRASQSVSSTYLTWYQQRPGQAPRLLIYGASSRATGIPDRFSGSGSGTDFTLTISRLEPEDVAVYYCQQGSAFPPTFGQGTKVEIKRAAA

SEQ ID NO: 119 - protein, 117 aa, synthetic construct
AEVQLVESGGGLVQPGGSLRLPCAASGFTFSNYVMHWVRQAPGKGLEWVAVISYDGSNKYYADSVKGRFTISRDNSKNTLYLQMNSLRAEDTAVYYCAKSHSNMSFDYWGQGTLVTV

SEQ ID NO: 120 - protein, 110 aa, synthetic construct
SELTQSPSSLSASVGDRVTITCRASQSISSYLNWYQQKPGKAPKLLIYAASSLQSGVPSRFSGSGSGTDFTLTISSLQPEDFATYYCQQSYSTPPTFGQGTKVEIKRAAA

SEQ ID NO: 121 - protein, 120 aa, synthetic construct
AQVQLVQSGPEVKKPGASVKVSCKASGYTFTSYYMHWVRQAPGQGLEWMGIINPSGGSTSYAQKFQGRVTMTRDTSTSTVYMELSSLRSEDAAVYYCARDYVRTSHSGFDYWGQGTLVTV

SEQ ID NO: 122 - protein, 112 aa, synthetic construct
SEIELTQSPSSLSASVGDRVTITCRASQSISSYLNWYQQKPGKAPKLLIYAASSLQSGVPSRFSGSGSGTDFTLTISSLQPEDFATYYCQQSYSTPPTFGQGTKVEIKRAAA

SEQ ID NO: 123 - protein, 121 aa, synthetic construct
AQVQLVQSGAEVKKPGASVKVSCKASGYTFTSYYMHWVRQAPGQGLEWMGIINPSGGGTSYAQKFQGRVTMTRDTSTSTVYMELSSLRSEDTAVYYCARDYYVTYDSWFDSWGQGTLVTVS

SEQ ID NO: 124 - protein, 111 aa, synthetic construct
SELTQDPAVSVALGQTVRITCQGDSLRSYYASWYQQKPGQAPVLVIYGKNNRPSGIPDRFSGSSSGNTASLTITGAQAEDEADYYCNSRDSSGNHVVFGGGTKLTVLGAAA

SEQ ID NO: 125 - protein, 117 aa, synthetic construct
AEVQLVESGGGLVQPGGSLRLPCAASGFTFSNYVMHWVRQAPGKGLEWVAVISYDGSNKYYADSVKGRFTISRDNSKNTLYLQMNSLRAEDTAVYYCAKSHSNMAFDYWGQGTLVTV

SEQ ID NO: 126 - protein, 110 aa, synthetic construct; identical to SEQ ID NO: 120

SEQ ID NO: 127 - protein, 120 aa, synthetic construct
AQVQLVQSGAEVKKPGASVKVSCKASGYTFTSYYMHWVRQAPGQGLEWMGIINPSGGSTSYAQKFQGRVTMTRDTSTSTVYMELSSLRSEDTAVYYCARDYQLSMTSGFDYWGQGTLVTV

SEQ ID NO: 128 - protein, 112 aa, synthetic construct; identical to SEQ ID NO: 122

SEQ ID NO: 129 - protein, 117 aa, synthetic construct
AEVQLVESGGGLVQPGGSLRLPCAASGFTFSNYVMHWVRQAPGKGLEWVAVISYDGSNKYYADSVKGRFTISRDNSKNTLYLQMNSLRAEDTAVYYCVKSHSNMAFDYWGQGTLVTV

SEQ ID NO: 130 - protein, 110 aa, synthetic construct; identical to SEQ ID NO: 120

SEQ ID NO: 131 - protein, 244 aa, synthetic construct
AEVQLVESGGGLVQPGGSLRLSCAASGFTFSGYLMSWVRQAPGKGLEWVAVISYDGSNKYYADSVKGRFTISRDNSKNTLYLQMDSLRAEDTAVYYCARARRDTNLFDYWGQGTLVTVLEGTGGSGGTGSGTGTSELTQSPSSLSASVGDRVTITCRASQSISSYLNWYQQKPGKAPKLLIYAASSLQSGVPSRFSGSGSGTDFTLTISSLQPEDFATYYCQQSYSTPPTFGQGTKVEIKRAAA

SEQ ID NO: 132 - protein, 248 aa, synthetic construct
AQVQLVQSGAEVKKPGASVKVSCKASGYTFTSYYMHWVRQAPGQGLEWMGIINPSGGGTSYAQKFQGRVTMTRDTSTSTVYMELSSLRSEDTAVYYCARDYYVTYDSWFDSWGQGTLVTVSRGGGGSGGGGSGGGGSSELTQDPAVSVALGQTVRITCQGDSLRSYYASWYQQKPGQAPVLVIYGKNNRPSGIPDRFSGSSSGNTASLTITGAQAEDEADYYCNSRDSSGNHVVFGGGTKLTVLGAAA

SEQ ID NO: 133 - protein, 253 aa, synthetic construct
SELDIQMTQSPPTLSLSPGERATLSCRASQSVSSTYLTWYQQRPGQAPRLLIYGASSRATGIPDRFSGSGSGTDFTLTISRLEPEDVAVYYCQQGSAFPPTFGQGTKVEIKRAAAGSTSGSGKPGSGEGSTKGAEVQLVESGGGVVQPGRSLRLSCAASGFTFSDYTMSWVRQAPGKGLEWVAVISYDGSNKYYADSVKGRFTISRDNSKNTLYLQMNSLRAEDTAVYYCAKDRGSAQGYPLDYWGQGTLVTV

SEQ ID NO: 134 - protein, 253 aa, synthetic construct
AEVQLVESGGGVVQPGRSLRLSCAASGFTFSDYTMSWVRQAPGKGLEWVAVISYDGSNKYYADSVKGRFTISRDNSKNTLYLQMNSLRAEDTAVYYCAKDRGSAQGYPLDYWGQGTLVTVGSTSGSGKPGSGEGSTKGSELDIQMTQSPPTLSLSPGERATLSCRASQSVSSTYLTWYQQRPGQAPRLLIYGASSRATGIPDRFSGSGSGTDFTLTISRLEPEDVAVYYCQQGSAFPPTFGQGTKVEIKRAAA

SEQ ID NO: 135 - protein, 245 aa, synthetic construct
SELTQSPSSLSASVGDRVTITCRASQSISSYLNWYQQKPGKAPKLLIYAASSLQSGVPSRFSGSGSGTDFTLTISSLQPEDFATYYCQQSYSTPPTFGQGTKVEIKRAAAGSTSGSGKPGSGEGSTKGAEVQLVESGGGLVQPGGSLRLPCAASGFTFSNYVMHWVRQAPGKGLEWVAVISYDGSNKYYADSVKGRFTISRDNSKNTLYLQMNSLRAEDTAVYYCAKSHSNMSFDYWGQGTLVTV

SEQ ID NO: 136 - protein, 245 aa, synthetic construct
AEVQLVESGGGLVQPGGSLRLPCAASGFTFSNYVMHWVRQAPGKGLEWVAVISYDGSNKYYADSVKGRFTISRDNSKNTLYLQMNSLRAEDTAVYYCAKSHSNMSFDYWGQGTLVTVGSTSGSGKPGSGEGSTKGSELTQSPSSLSASVGDRVTITCRASQSISSYLNWYQQKPGKAPKLLIYAASSLQSGVPSRFSGSGSGTDFTLTISSLQPEDFATYYCQQSYSTPPTFGQGTKVEIKRAAA

SEQ ID NO: 137 - protein, 246 aa, synthetic construct
SELTQSPSSLSASVGDRVTITCRASQSISSYLNWYQQKPGKAPKLLIYAASSLQSGVPSRFSGSGSGTDFTLTISSLQPEDFATYYCQQSYSTPPTFGQGTKVEIKRAAAGSTSGSGKPGSGEGSTKGAEVQLVESGGGLVQPGGSLRLSCAASGFTFSGYLMSWVRQAPGKGLEWVAVISYDGSNKYYADSVKGRFTISRDNSKNTLYLQMDSLRAEDTAVYYCARARRDTNLFDYWGQGTLVTV

SEQ ID NO: 138 - protein, 246 aa, synthetic construct
AEVQLVESGGGLVQPGGSLRLSCAASGFTFSGYLMSWVRQAPGKGLEWVAVISYDGSNKYYADSVKGRFTISRDNSKNTLYLQMDSLRAEDTAVYYCARARRDTNLFDYWGQGTLVTVGSTSGSGKPGSGEGSTKGSELTQSPSSLSASVGDRVTITCRASQSISSYLNWYQQKPGKAPKLLIYAASSLQSGVPSRFSGSGSGTDFTLTISSLQPEDFATYYCQQSYSTPPTFGQGTKVEIKRAAA

SEQ ID NO: 139 - protein, 250 aa, synthetic construct
SEIELTQSPSSLSASVGDRVTITCRASQSISSYLNWYQQKPGKAPKLLIYAASSLQSGVPSRFSGSGSGTDFTLTISSLQPEDFATYYCQQSYSTPPTFGQGTKVEIKRAAAGSTSGSGKPGSGEGSTKGAQVQLVQSGPEVKKPGASVKVSCKASGYTFTSYYMHWVRQAPGQGLEWMGIINPSGGSTSYAQKFQGRVTMTRDTSTSTVYMELSSLRSEDAAVYYCARDYVRTSHSGFDYWGQGTLVTV

SEQ ID NO: 140 - protein, 250 aa, synthetic construct
AQVQLVQSGPEVKKPGASVKVSCKASGYTFTSYYMHWVRQAPGQGLEWMGIINPSGGSTSYAQKFQGRVTMTRDTSTSTVYMELSSLRSEDAAVYYCARDYVRTSHSGFDYWGQGTLVTVGSTSGSGKPGSGEGSTKGSEIELTQSPSSLSASVGDRVTITCRASQSISSYLNWYQQKPGKAPKLLIYAASSLQSGVPSRFSGSGSGTDFTLTISSLQPEDFATYYCQQSYSTPPTFGQGTKVEIKRAAA

SEQ ID NO: 141 - protein, 250 aa, synthetic construct
SELTQDPAVSVALGQTVRITCQGDSLRSYYASWYQQKPGQAPVLVIYGKNNRPSGIPDRFSGSSSGNTASLTITGAQAEDEADYYCNSRDSSGNHVVFGGGTKLTVLGAAAGSTSGSGKPGSGEGSTKGAQVQLVQSGAEVKKPGASVKVSCKASGYTFTSYYMHWVRQAPGQGLEWMGIINPSGGGTSYAQKFQGRVTMTRDTSTSTVYMELSSLRSEDTAVYYCARDYYVTYDSWFDSWGQGTLVTVS

SEQ ID NO: 142 - protein, 250 aa, synthetic construct
AQVQLVQSGAEVKKPGASVKVSCKASGYTFTSYYMHWVRQAPGQGLEWMGIINPSGGGTSYAQKFQGRVTMTRDTSTSTVYMELSSLRSEDTAVYYCARDYYVTYDSWFDSWGQGTLVTVSGSTSGSGKPGSGEGSTKGSELTQDPAVSVALGQTVRITCQGDSLRSYYASWYQQKPGQAPVLVIYGKNNRPSGIPDRFSGSSSGNTASLTITGAQAEDEADYYCNSRDSSGNHVVFGGGTKLTVLGAAA

SEQ ID NO: 143 - protein, 245 aa, synthetic construct
SELTQSPSSLSASVGDRVTITCRASQSISSYLNWYQQKPGKAPKLLIYAASSLQSGVPSRFSGSGSGTDFTLTISSLQPEDFATYYCQQSYSTPPTFGQGTKVEIKRAAAGSTSGSGKPGSGEGSTKGAEVQLVESGGGLVQPGGSLRLPCAASGFTFSNYVMHWVRQAPGKGLEWVAVISYDGSNKYYADSVKGRFTISRDNSKNTLYLQMNSLRAEDTAVYYCAKSHSNMAFDYWGQGTLVTV

SEQ ID NO: 144 - protein, 245 aa, synthetic construct
AEVQLVESGGGLVQPGGSLRLPCAASGFTFSNYVMHWVRQAPGKGLEWVAVISYDGSNKYYADSVKGRFTISRDNSKNTLYLQMNSLRAEDTAVYYCAKSHSNMAFDYWGQGTLVTVGSTSGSGKPGSGEGSTKGSELTQSPSSLSASVGDRVTITCRASQSISSYLNWYQQKPGKAPKLLIYAASSLQSGVPSRFSGSGSGTDFTLTISSLQPEDFATYYCQQSYSTPPTFGQGTKVEIKRAAA

SEQ ID NO: 145 - protein, 250 aa, synthetic construct
SEIELTQSPSSLSASVGDRVTITCRASQSISSYLNWYQQKPGKAPKLLIYAASSLQSGVPSRFSGSGSGTDFTLTISSLQPEDFATYYCQQSYSTPPTFGQGTKVEIKRAAAGSTSGSGKPGSGEGSTKGAQVQLVQSGAEVKKPGASVKVSCKASGYTFTSYYMHWVRQAPGQGLEWMGIINPSGGSTSYAQKFQGRVTMTRDTSTSTVYMELSSLRSEDTAVYYCARDYQLSMTSGFDYWGQGTLVTV

SEQ ID NO: 146 - protein, 250 aa, synthetic construct
AQVQLVQSGAEVKKPGASVKVSCKASGYTFTSYYMHWVRQAPGQGLEWMGIINPSGGSTSYAQKFQGRVTMTRDTSTSTVYMELSSLRSEDTAVYYCARDYQLSMTSGFDYWGQGTLVTVGSTSGSGKPGSGEGSTKGSEIELTQSPSSLSASVGDRVTITCRASQSISSYLNWYQQKPGKAPKLLIYAASSLQSGVPSRFSGSGSGTDFTLTISSLQPEDFATYYCQQSYSTPPTFGQGTKVEIKRAAA

SEQ ID NO: 147 - protein, 245 aa, synthetic construct
SELTQSPSSLSASVGDRVTITCRASQSISSYLNWYQQKPGKAPKLLIYAASSLQSGVPSRFSGSGSGTDFTLTISSLQPEDFATYYCQQSYSTPPTFGQGTKVEIKRAAAGSTSGSGKPGSGEGSTKGAEVQLVESGGGLVQPGGSLRLPCAASGFTFSNYVMHWVRQAPGKGLEWVAVISYDGSNKYYADSVKGRFTISRDNSKNTLYLQMNSLRAEDTAVYYCVKSHSNMAFDYWGQGTLVTV

SEQ ID NO: 148 - protein, 245 aa, synthetic construct
AEVQLVESGGGLVQPGGSLRLPCAASGFTFSNYVMHWVRQAPGKGLEWVAVISYDGSNKYYADSVKGRFTISRDNSKNTLYLQMNSLRAEDTAVYYCVKSHSNMAFDYWGQGTLVTVGSTSGSGKPGSGEGSTKGSELTQSPSSLSASVGDRVTITCRASQSISSYLNWYQQKPGKAPKLLIYAASSLQSGVPSRFSGSGSGTDFTLTISSLQPEDFATYYCQQSYSTPPTFGQGTKVEIKRAAA

SEQ ID NO: 149 - protein, 251 aa, synthetic construct
SELDIQMTQSPPTLSLSPGERATLSCRASQSVSSTYLTWYQQRPGQAPRLLIYGASSRATGIPDRFSGSGSGTDFTLTISRLEPEDVAVYYCQQGSAFPPTFGQGTKVEIKRAAALEGTGGSGGTGSGTGTAEVQLVESGGGVVQPGRSLRLSCAASGFTFSDYTMSWVRQAPGKGLEWVAVISYDGSNKYYADSVKGRFTISRDNSKNTLYLQMNSLRAEDTAVYYCAKDRGSAQGYPLDYWGQGTLVTV

SEQ ID NO: 150 - protein, 251 aa, synthetic construct
AEVQLVESGGGVVQPGRSLRLSCAASGFTFSDYTMSWVRQAPGKGLEWVAVISYDGSNKYYADSVKGRFTISRDNSKNTLYLQMNSLRAEDTAVYYCAKDRGSAQGYPLDYWGQGTLVTVLEGTGGSGGTGSGTGTSELDIQMTQSPPTLSLSPGERATLSCRASQSVSSTYLTWYQQRPGQAPRLLIYGASSRATGIPDRFSGSGSGTDFTLTISRLEPEDVAVYYCQQGSAFPPTFGQGTKVEIKRAAA

SEQ ID NO: 151 - protein, 243 aa, synthetic construct
SELTQSPSSLSASVGDRVTITCRASQSISSYLNWYQQKPGKAPKLLIYAASSLQSGVPSRFSGSGSGTDFTLTISSLQPEDFATYYCQQSYSTPPTFGQGTKVEIKRAAALEGTGGSGGTGSGTGTAEVQLVESGGGLVQPGGSLRLPCAASGFTFSNYVMHWVRQAPGKGLEWVAVISYDGSNKYYADSVKGRFTISRDNSKNTLYLQMNSLRAEDTAVYYCAKSHSNMSFDYWGQGTLVTV

SEQ ID NO: 152 - protein, 243 aa, synthetic construct
AEVQLVESGGGLVQPGGSLRLPCAASGFTFSNYVMHWVRQAPGKGLEWVAVISYDGSNKYYADSVKGRFTISRDNSKNTLYLQMNSLRAEDTAVYYCAKSHSNMSFDYWGQGTLVTVLEGTGGSGGTGSGTGTSELTQSPSSLSASVGDRVTITCRASQSISSYLNWYQQKPGKAPKLLIYAASSLQSGVPSRFSGSGSGTDFTLTISSLQPEDFATYYCQQSYSTPPTFGQGTKVEIKRAAA

SEQ ID NO: 153 - protein, 244 aa, synthetic construct
SELTQSPSSLSASVGDRVTITCRASQSISSYLNWYQQKPGKAPKLLIYAASSLQSGVPSRFSGSGSGTDFTLTISSLQPEDFATYYCQQSYSTPPTFGQGTKVEIKRAAALEGTGGSGGTGSGTGTAEVQLVESGGGLVQPGGSLRLSCAASGFTFSGYLMSWVRQAPGKGLEWVAVISYDGSNKYYADSVKGRFTISRDNSKNTLYLQMDSLRAEDTAVYYCARARRDTNLFDYWGQGTLVTV

SEQ ID NO: 154 - protein, 244 aa, synthetic construct; identical to SEQ ID NO: 131

SEQ ID NO: 155 - protein, 248 aa, synthetic construct
SEIELTQSPSSLSASVGDRVTITCRASQSISSYLNWYQQKPGKAPKLLIYAASSLQSGVPSRFSGSGSGTDFTLTISSLQPEDFATYYCQQSYSTPPTFGQGTKVEIKRAAASSGGGGSGGGGSGGGGAQVQLVQSGPEVKKPGASVKVSCKASGYTFTSYYMHWVRQAPGQGLEWMGIINPSGGSTSYAQKFQGRVTMTRDTSTSTVYMELSSLRSEDAAVYYCARDYVRTSHSGFDYWGQGTLVTV

SEQ ID NO: 156 - protein, 248 aa, synthetic construct
AQVQLVQSGPEVKKPGASVKVSCKASGYTFTSYYMHWVRQAPGQGLEWMGIINPSGGSTSYAQKFQGRVTMTRDTSTSTVYMELSSLRSEDAAVYYCARDYVRTSHSGFDYWGQGTLVTVSSGGGGSGGGGSGGGGSEIELTQSPSSLSASVGDRVTITCRASQSISSYLNWYQQKPGKAPKLLIYAASSLQSGVPSRFSGSGSGTDFTLTISSLQPEDFATYYCQQSYSTPPTFGQGTKVEIKRAAA

SEQ ID NO: 157 - protein, 248 aa, synthetic construct
SELTQDPAVSVALGQTVRITCQGDSLRSYYASWYQQKPGQAPVLVIYGKNNRPSGIPDRFSGSSSGNTASLTITGAQAEDEADYYCNSRDSSGNHVVFGGGTKLTVLGAAARGGGGSGGGGSGGGGSAQVQLVQSGAEVKKPGASVKVSCKASGYTFTSYYMHWVRQAPGQGLEWMGIINPSGGGTSYAQKFQGRVTMTRDTSTSTVYMELSSLRSEDTAVYYCARDYYVTYDSWFDSWGQGTLVTVS

SEQ ID NO: 158 - protein, 248 aa, synthetic construct; identical to SEQ ID NO: 132

SEQ ID NO: 159 - protein, 243 aa, synthetic construct
SELTQSPSSLSASVGDRVTITCRASQSISSYLNWYQQKPGKAPKLLIYAASSLQSGVPSRFSGSGSGTDFTLTISSLQPEDFATYYCQQSYSTPPTFGQGTKVEIKRAAALEGTGGSGGTGSGTGTAEVQLVESGGGLVQPGGSLRLPCAASGFTFSNYVMHWVRQAPGKGLEWVAVISYDGSNKYYADSVKGRFTISRDNSKNTLYLQMNSLRAEDTAVYYCAKSHSNMAFDYWGQGTLVTV

SEQ ID NO: 160 - protein, 243 aa, synthetic construct
AEVQLVESGGGLVQPGGSLRLPCAASGFTFSNYVMHWVRQAPGKGLEWVAVISYDGSNKYYADSVKGRFTISRDNSKNTLYLQMNSLRAEDTAVYYCAKSHSNMAFDYWGQGTLVTVLEGTGGSGGTGSGTGTSELTQSPSSLSASVGDRVTITCRASQSISSYLNWYQQKPGKAPKLLIYAASSLQSGVPSRFSGSGSGTDFTLTISSLQPEDFATYYCQQSYSTPPTFGQGTKVEIKRAAA

SEQ ID NO: 161 - protein, 248 aa, synthetic construct
SEIELTQSPSSLSASVGDRVTITCRASQSISSYLNWYQQKPGKAPKLLIYAASSLQSGVPSRFSGSGSGTDFTLTISSLQPEDFATYYCQQSYSTPPTFGQGTKVEIKRAAASSGGGGSGGGGSGGGGAQVQLVQSGAEVKKPGASVKVSCKASGYTFTSYYMHWVRQAPGQGLEWMGIINPSGGSTSYAQKFQGRVTMTRDTSTSTVYMELSSLRSEDTAVYYCARDYQLSMTSGFDYWGQGTLVTV

SEQ ID NO: 162 - protein, 248 aa, synthetic construct
AQVQLVQSGAEVKKPGASVKVSCKASGYTFTSYYMHWVRQAPGQGLEWMGIINPSGGSTSYAQKFQGRVTMTRDTSTSTVYMELSSLRSEDTAVYYCARDYQLSMTSGFDYWGQGTLVTVSSGGGGSGGGGSGGGGSEIELTQSPSSLSASVGDRVTITCRASQSISSYLNWYQQKPGKAPKLLIYAASSLQSGVPSRFSGSGSGTDFTLTISSLQPEDFATYYCQQSYSTPPTFGQGTKVEIKRAAA

SEQ ID NO: 163 - protein, 243 aa, synthetic construct
SELTQSPSSLSASVGDRVTITCRASQSISSYLNWYQQKPGKAPKLLIYAASSLQSGVPSRFSGSGSGTDFTLTISSLQPEDFATYYCQQSYSTPPTFGQGTKVEIKRAAALEGTGGSGGTGSGTGTAEVQLVESGGGLVQPGGSLRLPCAASGFTFSNYVMHWVRQAPGKGLEWVAVISYDGSNKYYADSVKGRFTISRDNSKNTLYLQMNSLRAEDTAVYYCVKSHSNMAFDYWGQGTLVTV

SEQ ID NO: 164 - protein, 243 aa, synthetic construct
AEVQLVESGGGLVQPGGSLRLPCAASGFTFSNYVMHWVRQAPGKGLEWVAVISYDGSNKYYADSVKGRFTISRDNSKNTLYLQMNSLRAEDTAVYYCVKSHSNMAFDYWGQGTLVTVLEGTGGSGGTGSGTGTSELTQSPSSLSASVGDRVTITCRASQSISSYLNWYQQKPGKAPKLLIYAASSLQSGVPSRFSGSGSGTDFTLTISSLQPEDFATYYCQQSYSTPPTFGQGTKVEIKRAAA

SEQ ID NO: 165 - protein, 15 aa, synthetic construct
GGGGSGGGGSGGGGS

SEQ ID NO: 166 - protein, 15 aa, synthetic construct
GTGGSGGTGSGTGTS

SEQ ID NO: 167 - protein, 18 aa, synthetic construct
GSTSGSGKPGSGEGSTKG

SEQ ID NO: 168 - protein, 16 aa, synthetic construct
LEGTGGSGGTGSGTGT

SEQ ID NO: 169 - protein, 16 aa, synthetic construct
SSGGGGSGGGGSGGGG

SEQ ID NO: 170 - protein, 16 aa, synthetic construct
RGGGGSGGGGSGGGGS

SEQ ID NO: 171 - protein, 12 aa, synthetic construct
ESKYGPPCPPCP

SEQ ID NO: 172 - protein, 45 aa, synthetic construct
TTTPAPRPPTPAPTIASQPLSLRPEACRPAAGGAVHTRGLDFACD

SEQ ID NO: 173 - protein, 39 aa, synthetic construct; identical to SEQ ID NO: 10

SEQ ID NO: 174 - protein, 24 aa, synthetic construct
IYIWAPLAGTCGVLLLSLVITLYC

SEQ ID NO: 175 - protein, 27 aa, synthetic construct
FWVLVVVGGVLACYSLLVTVAFIIFWV

SEQ ID NO: 176 - protein, 28 aa, synthetic construct
MFWVLVVVGGVLACYSLLVTVAFIIFWV

SEQ ID NO: 177 - protein, 113 aa, synthetic construct; identical to SEQ ID NO: 14

SEQ ID NO: 178 - protein, 112 aa, synthetic construct; identical to SEQ ID NO: 15

SEQ ID NO: 179 - protein, 41 aa, synthetic construct; identical to SEQ ID NO: 12

SEQ ID NO: 180 - protein, 41 aa, synthetic construct; identical to SEQ ID NO: 13

SEQ ID NO: 181 - protein, 42 aa, synthetic construct
KRGRKKLLYIFKQPFMRPVQTTQEEDGCSCRFPEEEEGGCEL

SEQ ID NO: 182 - protein, 458 aa, synthetic construct
MLLVTSLLLCELPHPAFLLIPAEVQLVESGGGLVQPGGSLRLSCAASGFTFSGYLMSWVRQAPGKGLEWVAVISYDGSNKYYADSVKGRFTISRDNSKNTLYLQMDSLRAEDTAVYYCARARRDTNLFDYWGQGTLVTVLEGTGGSGGTGSGTGTSELTQSPSSLSASVGDRVTITCRASQSISSYLNWYQQKPGKAPKLLIYAASSLQSGVPSRFSGSGSGTDFTLTISSLQPEDFATYYCQQSYSTPPTFGQGTKVEIKRAAAESKYGPPCPPCPFWVLVVVGGVLACYSLLVTVAFIIFWVRSKRSRLLHSDYMNMTPRRPGPTRKHYQPYAPPRDFAAYRSRVKFSRSADAPAYQQGQNQLYNELNLGRREEYDVLDKRRGRDPEMGGKPQRRKNPQEGLYNELQKDKMAEAYSEIGMKGERRRGKGHDGLYQGLSTATKDTYDALHMQALPPR

SEQ ID NO: 183 - protein, 462 aa, synthetic construct
MLLVTSLLLCELPHPAFLLIPAQVQLVQSGAEVKKPGASVKVSCKASGYTFTSYYMHWVRQAPGQGLEWMGIINPSGGGTSYAQKFQGRVTMTRDTSTSTVYMELSSLRSEDTAVYYCARDYYVTYDSWFDSWGQGTLVTVSRGGGGSGGGGSGGGGSSELTQDPAVSVALGQTVRITCQGDSLRSYYASWYQQKPGQAPVLVIYGKNNRPSGIPDRFSGSSSGNTASLTITGAQAEDEADYYCNSRDSSGNHVVFGGGTKLTVLGAAAESKYGPPCPPCPFWVLVVVGGVLACYSLLVTVAFIIFWVRSKRSRLLHSDYMNMTPRRPGPTRKHYQPYAPPRDFAAYRSRVKFSRSADAPAYQQGQNQLYNELNLGRREEYDVLDKRRGRDPEMGGKPQRRKNPQEGLYNELQKDKMAEAYSEIGMKGERRRGKGHDGLYQGLSTATKDTYDALHMQALPPR

SEQ ID NO: 184 - protein, 459 aa, synthetic construct
MLLVTSLLLCELPHPAFLLIPAEVQLVESGGGLVQPGGSLRLSCAASGFTFSGYLMSWVRQAPGKGLEWVAVISYDGSNKYYADSVKGRFTISRDNSKNTLYLQMDSLRAEDTAVYYCARARRDTNLFDYWGQGTLVTVLEGTGGSGGTGSGTGTSELTQSPSSLSASVGDRVTITCRASQSISSYLNWYQQKPGKAPKLLIYAASSLQSGVPSRFSGSGSGTDFTLTISSLQPEDFATYYCQQSYSTPPTFGQGTKVEIKRAAAESKYGPPCPPCPFWVLVVVGGVLACYSLLVTVAFIIFWVKRGRKKLLYIFKQPFMRPVQTTQEEDGCSCRFPEEEEGGCELRVKFSRSADAPAYQQGQNQLYNELNLGRREEYDVLDKRRGRDPEMGGKPQRRKNPQEGLYNELQKDKMAEAYSEIGMKGERRRGKGHDGLYQGLSTATKDTYDALHMQALPPR

SEQ ID NO: 185 - protein, 463 aa, synthetic construct
MLLVTSLLLCELPHPAFLLIPAQVQLVQSGAEVKKPGASVKVSCKASGYTFTSYYMHWVRQAPGQGLEWMGIINPSGGGTSYAQKFQGRVTMTRDTSTSTVYMELSSLRSEDTAVYYCARDYYVTYDSWFDSWGQGTLVTVSRGGGGSGGGGSGGGGSSELTQDPAVSVALGQTVRITCQGDSLRSYYASWYQQKPGQAPVLVIYGKNNRPSGIPDRFSGSSSGNTASLTITGAQAEDEADYYCNSRDSSGNHVVFGGGTKLTVLGAAAESKYGPPCPPCPFWVLVVVGGVLACYSLLVTVAFIIFWVKRGRKKLLYIFKQPFMRPVQTTQEEDGCSCRFPEEEEGGCELRVKFSRSADAPAYQQGQNQLYNELNLGRREEYDVLDKRRGRDPEMGGKPQRRKNPQEGLYNELQKDKMAEAYSEIGMKGERRRGKGHDGLYQGLSTATKDTYDALHMQALPPR

SEQ ID NO: 186 - protein, 485 aa, synthetic construct
MLLVTSLLLCELPHPAFLLIPAEVQLVESGGGLVQPGGSLRLSCAASGFTFSGYLMSWVRQAPGKGLEWVAVISYDGSNKYYADSVKGRFTISRDNSKNTLYLQMDSLRAEDTAVYYCARARRDTNLFDYWGQGTLVTVLEGTGGSGGTGSGTGTSELTQSPSSLSASVGDRVTITCRASQSISSYLNWYQQKPGKAPKLLIYAASSLQSGVPSRFSGSGSGTDFTLTISSLQPEDFATYYCQQSYSTPPTFGQGTKVEIKRAAAIEVMYPPPYLDNEKSNGTIIHVKGKHLCPSPLFPGPSKPFWVLVVVGGVLACYSLLVTVAFIIFWVRSKRSRLLHSDYMNMTPRRPGPTRKHYQPYAPPRDFAAYRSRVKFSRSADAPAYQQGQNQLYNELNLGRREEYDVLDKRRGRDPEMGGKPQRRKNPQEGLYNELQKDKMAEAYSEIGMKGERRRGKGHDGLYQGLSTATKDTYDALHMQALPPR

SEQ ID NO: 187 - protein, 489 aa, synthetic construct
MLLVTSLLLCELPHPAFLLIPAQVQLVQSGAEVKKPGASVKVSCKASGYTFTSYYMHWVRQAPGQGLEWMGIINPSGGGTSYAQKFQGRVTMTRDTSTSTVYMELSSLRSEDTAVYYCARDYYVTYDSWFDSWGQGTLVTVSRGGGGSGGGGSGGGGSSELTQDPAVSVALGQTVRITCQGDSLRSYYASWYQQKPGQAPVLVIYGKNNRPSGIPDRFSGSSSGNTASLTITGAQAEDEADYYCNSRDSSGNHVVFGGGTKLTVLGAAAIEVMYPPPYLDNEKSNGTIIHVKGKHLCPSPLFPGPSKPFWVLVVVGGVLACYSLLVTVAFIIFWVRSKRSRLLHSDYMNMTPRRPGPTRKHYQPYAPPRDFAAYRSRVKFSRSADAPAYQQGQNQLYNELNLGRREEYDVLDKRRGRDPEMGGKPQRRKNPQEGLYNELQKDKMAEAYSEIGMKGERRRGKGHDGLYQGLSTATKDTYDALHMQALPPR

SEQ ID NO: 188 - protein, 486 aa, synthetic construct
MLLVTSLLLCELPHPAFLLIPAEVQLVESGGGLVQPGGSLRLSCAASGFTFSGYLMSWVRQAPGKGLEWVAVISYDGSNKYYADSVKGRFTISRDNSKNTLYLQMDSLRAEDTAVYYCARARRDTNLFDYWGQGTLVTVLEGTGGSGGTGSGTGTSELTQSPSSLSASVGDRVTITCRASQSISSYLNWYQQKPGKAPKLLIYAASSLQSGVPSRFSGSGSGTDFTLTISSLQPEDFATYYCQQSYSTPPTFGQGTKVEIKRAAAIEVMYPPPYLDNEKSNGTIIHVKGKHLCPSPLFPGPSKPFWVLVVVGGVLACYSLLVTVAFIIFWVKRGRKKLLYIFKQPFMRPVQTTQEEDGCSCRFPEEEEGGCELRVKFSRSADAPAYQQGQNQLYNELNLGRREEYDVLDKRRGRDPEMGGKPQRRKNPQEGLYNELQKDKMAEAYSEIGMKGERRRGKGHDGLYQGLSTATKDTYDALHMQALPPR

SEQ ID NO: 189 - protein, 490 aa, synthetic construct
MLLVTSLLLCELPHPAFLLIPAQVQLVQSGAEVKKPGASVKVSCKASGYTFTSYYMHWVRQAPGQGLEWMGIINPSGGGTSYAQKFQGRVTMTRDTSTSTVYMELSSLRSEDTAVYYCARDYYVTYDSWFDSWGQGTLVTVSRGGGGSGGGGSGGGGSSELTQDPAVSVALGQTVRITCQGDSLRSYYASWYQQKPGQAPVLVIYGKNNRPSGIPDRFSGSSSGNTASLTITGAQAEDEADYYCNSRDSSGNHVVFGGGTKLTVLGAAAIEVMYPPPYLDNEKSNGTIIHVKGKHLCPSPLFPGPSKPFWVLVVVGGVLACYSLLVTVAFIIFWVKRGRKKLLYIFKQPFMRPVQTTQEEDGCSCRFPEEEEGGCELRVKFSRSADAPAYQQGQNQLYNELNLGRREEYDVLDKRRGRDPEMGGKPQRRKNPQEGLYNELQKDKMAEAYSEIGMKGERRRGKGHDGLYQGLSTATKDTYDALHMQALPPR

SEQ ID NO: 190 - protein, 455 aa, synthetic construct
MLLVTSLLLCELPHPAFLLIPAEVQLVESGGGLVQPGGSLRLSCAASGFTFSGYLMSWVRQAPGKGLEWVAVISYDGSNKYYADSVKGRFTISRDNSKNTLYLQMDSLRAEDTAVYYCARARRDTNLFDYWGQGTLVTVLEGTGGSGGTGSGTGTSELTQSPSSLSASVGDRVTITCRASQSISSYLNWYQQKPGKAPKLLIYAASSLQSGVPSRFSGSGSGTDFTLTISSLQPEDFATYYCQQSYSTPPTFGQGTKVEIKRAAAESKYGPPCPPCPIYIWAPLAGTCGVLLLSLVITLYCRSKRSRLLHSDYMNMTPRRPGPTRKHYQPYAPPRDFAAYRSRVKFSRSADAPAYQQGQNQLYNELNLGRREEYDVLDKRRGRDPEMGGKPQRRKNPQEGLYNELQKDKMAEAYSEIGMKGERRRGKGHDGLYQGLSTATKDTYDALHMQALPPR

SEQ ID NO: 191 - protein, 459 aa, synthetic construct
MLLVTSLLLCELPHPAFLLIPAQVQLVQSGAEVKKPGASVKVSCKASGYTFTSYYMHWVRQAPGQGLEWMGIINPSGGGTSYAQKFQGRVTMTRDTSTSTVYMELSSLRSEDTAVYYCARDYYVTYDSWFDSWGQGTLVTVSRGGGGSGGGGSGGGGSSELTQDPAVSVALGQTVRITCQGDSLRSYYASWYQQKPGQAPVLVIYGKNNRPSGIPDRFSGSSSGNTASLTITGAQAEDEADYYCNSRDSSGNHVVFGGGTKLTVLGAAAESKYGPPCPPCPIYIWAPLAGTCGVLLLSLVITLYCRSKRSRLLHSDYMNMTPRRPGPTRKHYQPYAPPRDFAAYRSRVKFSRSADAPAYQQGQNQLYNELNLGRREEYDVLDKRRGRDPEMGGKPQRRKNPQEGLYNELQKDKMAEAYSEIGMKGERRRGKGHDGLYQGLSTATKDTYDALHMQALPPR

SEQ ID NO: 192 - protein, 488 aa, synthetic construct
MLLVTSLLLCELPHPAFLLIPAEVQLVESGGGLVQPGGSLRLSCAASGFTFSGYLMSWVRQAPGKGLEWVAVISYDGSNKYYADSVKGRFTISRDNSKNTLYLQMDSLRAEDTAVYYCARARRDTNLFDYWGQGTLVTVLEGTGGSGGTGSGTGTSELTQSPSSLSASVGDRVTITCRASQSISSYLNWYQQKPGKAPKLLIYAASSLQSGVPSRFSGSGSGTDFTLTISSLQPEDFATYYCQQSYSTPPTFGQGTKVEIKRAAATTTPAPRPPTPAPTIASQPLSLRPEACRPAAGGAVHTRGLDFACDIYIWAPLAGTCGVLLLSLVITLYCRSKRSRLLHSDYMNMTPRRPGPTRKHYQPYAPPRDFAAYRSRVKFSRSADAPAYQQGQNQLYNELNLGRREEYDVLDKRRGRDPEMGGKPQRRKNPQEGLYNELQKDKMAEAYSEIGMKGERRRGKGHDGLYQGLSTATKDTYDALHMQALPPR

SEQ ID NO: 193 - protein, 492 aa, synthetic construct
MLLVTSLLLCELPHPAFLLIPAQVQLVQSGAEVKKPGASVKVSCKASGYTFTSYYMHWVRQAPGQGLEWMGIINPSGGGTSYAQKFQGRVTMTRDTSTSTVYMELSSLRSEDTAVYYCARDYYVTYDSWFDSWGQGTLVTVSRGGGGSGGGGSGGGGSSELTQDPAVSVALGQTVRITCQGDSLRSYYASWYQQKPGQAPVLVIYGKNNRPSGIPDRFSGSSSGNTASLTITGAQAEDEADYYCNSRDSSGNHVVFGGGTKLTVLGAAATTTPAPRPPTPAPTIASQPLSLRPEACRPAAGGAVHTRGLDFACDIYIWAPLAGTCGVLLLSLVITLYCRSKRSRLLHSDYMNMTPRRPGPTRKHYQPYAPPRDFAAYRSRVKFSRSADAPAYQQGQNQLYNELNLGRREEYDVLDKRRGRDPEMGGKPQRRKNPQEGLYNELQKDKMAEAYSEIGMKGERRRGKGHDGLYQGLSTATKDTYDALHMQALPPR

SEQ ID NO: 194 - protein, 456 aa, synthetic construct
MLLVTSLLLCELPHPAFLLIPAEVQLVESGGGLVQPGGSLRLSCAASGFTFSGYLMSWVRQAPGKGLEWVAVISYDGSNKYYADSVKGRFTISRDNSKNTLYLQMDSLRAEDTAVYYCARARRDTNLFDYWGQGTLVTVLEGTGGSGGTGSGTGTSELTQSPSSLSASVGDRVTITCRASQSISSYLNWYQQKPGKAPKLLIYAASSLQSGVPSRFSGSGSGTDFTLTISSLQPEDFATYYCQQSYSTPPTFGQGTKVEIKRAAAESKYGPPCPPCPIYIWAPLAGTCGVLLLSLVITLYCKRGRKKLLYIFKQPFMRPVQTTQEEDGCSCRFPEEEEGGCELRVKFSRSADAPAYQQGQNQLYNELNLGRREEYDVLDKRRGRDPEMGGKPQRRKNPQEGLYNELQKDKMAEAYSEIGMKGERRRGKGHDGLYQGLSTATKDTYDALHMQALPPR

SEQ ID NO: 195 - protein, 460 aa, synthetic construct
MLLVTSLLLCELPHPAFLLIPAQVQLVQSGAEVKKPGASVKVSCKASGYTFTSYYMHWVRQAPGQGLEWMGIINPSGGGTSYAQKFQGRVTMTRDTSTSTVYMELSSLRSEDTAVYYCARDYYVTYDSWFDSWGQGTLVTVSRGGGGSGGGGSGGGGSSELTQDPAVSVALGQTVRITCQGDSLRSYYASWYQQKPGQAPVLVIYGKNNRPSGIPDRFSGSSSGNTASLTITGAQAEDEADYYCNSRDSSGNHVVFGGGTKLTVLGAAAESKYGPPCPPCPIYIWAPLAGTCGVLLLSLVITLYCKRGRKKLLYIFKQPFMRPVQTTQEEDGCSCRFPEEEEGGCELRVKFSRSADAPAYQQGQNQLYNELNLGRREEYDVLDKRRGRDPEMGGKPQRRKNPQEGLYNELQKDKMAEAYSEIGMKGERRRGKGHDGLYQGLSTATKDTYDALHMQALPPR

SEQ ID NO: 196 - protein, 489 aa, synthetic construct
MLLVTSLLLCELPHPAFLLIPAEVQLVESGGGLVQPGGSLRLSCAASGFTFSGYLMSWVRQAPGKGLEWVAVISYDGSNKYYADSVKGRFTISRDNSKNTLYLQMDSLRAEDTAVYYCARARRDTNLFDYWGQGTLVTVLEGTGGSGGTGSGTGTSELTQSPSSLSASVGDRVTITCRASQSISSYLNWYQQKPGKAPKLLIYAASSLQSGVPSRFSGSGSGTDFTLTISSLQPEDFATYYCQQSYSTPPTFGQGTKVEIKRAAATTTPAPRPPTPAPTIASQPLSLRPEACRPAAGGAVHTRGLDFACDIYIWAPLAGTCGVLLLSLVITLYCKRGRKKLLYIFKQPFMRPVQTTQEEDGCSCRFPEEEEGGCELRVKFSRSADAPAYQQGQNQLYNELNLGRREEYDVLDKRRGRDPEMGGKPQRRKNPQEGLYNELQKDKMAEAYSEIGMKGERRRGKGHDGLYQGLSTATKDTYDALHMQALPPR

SEQ ID NO: 197 - protein, 493 aa, synthetic construct
MLLVTSLLLCELPHPAFLLIPAQVQLVQSGAEVKKPGASVKVSCKASGYTFTSYYMHWVRQAPGQGLEWMGIINPSGGGTSYAQKFQGRVTMTRDTSTSTVYMELSSLRSEDTAVYYCARDYYVTYDSWFDSWGQGTLVTVSRGGGGSGGGGSGGGGSSELTQDPAVSVALGQTVRITCQGDSLRSYYASWYQQKPGQAPVLVIYGKNNRPSGIPDRFSGSSSGNTASLTITGAQAEDEADYYCNSRDSSGNHVVFGGGTKLTVLGAAATTTPAPRPPTPAPTIASQPLSLRPEACRPAAGGAVHTRGLDFACDIYIWAPLAGTCGVLLLSLVITLYCKRGRKKLLYIFKQPFMRPVQTTQEEDGCSCRFPEEEEGGCELRVKFSRSADAPAYQQGQNQLYNELNLGRREEYDVLDKRRGRDPEMGGKPQRRKNPQEGLYNELQKDKMAEAYSEIGMKGERRRGKGHDGLYQGLSTATKDTYDALHMQALPPR

SEQ ID NO: 198 - protein, 474 aa, synthetic construct
MLLLVTSLLLCELPHPAFLLIPEQKLISEEDLAQVQLVQSGAEVKKPGASVKVSCKASGYTFTSYYMHWVRQAPGQGLEWMGIINPSGGGTSYAQKFQGRVTMTRDTSTSTVYMELSSLRSEDTAVYYCARDYYVTYDSWFDSWGQGTLVTVSRGGGGSGGGGSGGGGSSELTQDPAVSVALGQTVRITCQGDSLRSYYASWYQQKPGQAPVLVIYGKNNRPSGIPDRFSGSSSGNTASLTITGAQAEDEADYYCNSRDSSGNHVVFGGGTKLTVLGAAAESKYGPPCPPCPMFWVLVVVGGVLACYSLLVTVAFIIFWVKRGRKKLLYIFKQPFMRPVQTTQEEDGCSCRFPEEEEGGCELRVKFSRSADAPAYQQGQNQLYNELNLGRREEYDVLDKRRGRDPEMGGKPRRKNPQEGLYNELQKDKMAEAYSEIGMKGERRRGKGHDGLYQGLSTATKDTYDALHMQALPPR

SEQ ID NO: 199 - protein, 472 aa, synthetic construct
MVLQTQVFISLLLWISGAYGEQKLISEEDLAQVQLVQSGAEVKKPGASVKVSCKASGYTFTSYYMHWVRQAPGQGLEWMGIINPSGGGTSYAQKFQGRVTMTRDTSTSTVYMELSSLRSEDTAVYYCARDYYVTYDSWFDSWGQGTLVTVSRGGGGSGGGGSGGGGSSELTQDPAVSVALGQTVRITCQGDSLRSYYASWYQQKPGQAPVLVIYGKNNRPSGIPDRFSGSSSGNTASLTITGAQAEDEADYYCNSRDSSGNHVVFGGGTKLTVLGAAAESKYGPPCPPCPMFWVLVVVGGVLACYSLLVTVAFIIFWVKRGRKKLLYIFKQPFMRPVQTTQEEDGCSCRFPEEEEGGCELRVKFSRSADAPAYQQGQNQLYNELNLGRREEYDVLDKRRGRDPEMGGKPRRKNPQEGLYNELQKDKMAEAYSEIGMKGERRRGKGHDGLYQGLSTATKDTYDALHMQALPPR

SEQ ID NO: 200 - protein, 470 aa, synthetic construct
MALPVTALLLPLALLLHAEQKLISEEDLAQVQLVQSGAEVKKPGASVKVSCKASGYTFTSYYMHWVRQAPGQGLEWMGIINPSGGGTSYAQKFQGRVTMTRDTSTSTVYMELSSLRSEDTAVYYCARDYYVTYDSWFDSWGQGTLVTVSRGGGGSGGGGSGGGGSSELTQDPAVSVALGQTVRITCQGDSLRSYYASWYQQKPGQAPVLVIYGKNNRPSGIPDRFSGSSSGNTASLTITGAQAEDEADYYCNSRDSSGNHVVFGGGTKLTVLGAAAESKYGPPCPPCPMFWVLVVVGGVLACYSLLVTVAFIIFWVKRGRKKLLYIFKQPFMRPVQTTQEEDGCSCRFPEEEEGGCELRVKFSRSADAPAYQQGQNQLYNELNLGRREEYDVLDKRRGRDPEMGGKPRRKNPQEGLYNELQKDKMAEAYSEIGMKGERRRGKGHDGLYQGLSTATKDTYDALHMQALPPR

SEQ ID NO: 201 - protein, 472 aa, synthetic construct
MYRMQLLSCIALSLALVTNSEQKLISEEDLAQVQLVQSGAEVKKPGASVKVSCKASGYTFTSYYMHWVRQAPGQGLEWMGIINPSGGGTSYAQKFQGRVTMTRDTSTSTVYMELSSLRSEDTAVYYCARDYYVTYDSWFDSWGQGTLVTVSRGGGGSGGGGSGGGGSSELTQDPAVSVALGQTVRITCQGDSLRSYYASWYQQKPGQAPVLVIYGKNNRPSGIPDRFSGSSSGNTASLTITGAQAEDEADYYCNSRDSSGNHVVFGGGTKLTVLGAAAESKYGPPCPPCPMFWVLVVVGGVLACYSLLVTVAFIIFWVKRGRKKLLYIFKQPFMRPVQTTQEEDGCSCRFPEEEEGGCELRVKFSRSADAPAYQQGQNQLYNELNLGRREEYDVLDKRRGRDPEMGGKPRRKNPQEGLYNELQKDKMAEAYSEIGMKGERRRGKGHDGLYQGLSTATKDTYDALHMQALPPR

SEQ ID NO: 202 - protein, 474 aa, synthetic construct; identical to SEQ ID NO: 198

SEQ ID NO: 203 - protein, 447 aa, synthetic construct
SELDIQMTQSPPTLSLSPGERATLSCRASQSVSSTYLTWYQQRPGQAPRLLIYGASSRATGIPDRFSGSGSGTDFTLTISRLEPEDVAVYYCQQGSAFPPTFGQGTKVEIKRAAAGSTSGSGKPGSGEGSTKGAEVQLVESGGGVVQPGRSLRLSCAASGFTFSDYTMSWVRQAPGKGLEWVAVISYDGSNKYYADSVKGRFTISRDNSKNTLYLQMNSLRAEDTAVYYCAKDRGSAQGYPLDYWGQGTLVTVESKYGPPCPPCPMFWVLVVVGGVLACYSLLVTVAFIIFWVKRGRKKLLYIFKQPFMRPVQTTQEEDGCSCRFPEEEEGGCELRVKFSRSADAPAYQQGQNQLYNELNLGRREEYDVLDKRRGRDPEMGGKPRRKNPQEGLYNELQKDKMAEAYSEIGMKGERRRGKGHDGLYQGLSTATKDTYDALHMQALPPR

SEQ ID NO: 204 - protein, 447 aa, synthetic construct
AEVQLVESGGGVVQPGRSLRLSCAASGFTFSDYTMSWVRQAPGKGLEWVAVISYDGSNKYYADSVKGRFTISRDNSKNTLYLQMNSLRAEDTAVYYCAKDRGSAQGYPLDYWGQGTLVTVGSTSGSGKPGSGEGSTKGSELDIQMTQSPPTLSLSPGERATLSCRASQSVSSTYLTWYQQRPGQAPRLLIYGASSRATGIPDRFSGSGSGTDFTLTISRLEPEDVAVYYCQQGSAFPPTFGQGTKVEIKRAAAESKYGPPCPPCPMFWVLVVVGGVLACYSLLVTVAFIIFWVKRGRKKLLYIFKQPFMRPVQTTQEEDGCSCRFPEEEEGGCELRVKFSRSADAPAYQQGQNQLYNELNLGRREEYDVLDKRRGRDPEMGGKPRRKNPQEGLYNELQKDKMAEAYSEIGMKGERRRGKGHDGLYQGLSTATKDTYDALHMQALPPR

SEQ ID NO: 205 - protein, 439 aa, synthetic construct
SELTQSPSSLSASVGDRVTITCRASQSISSYLNWYQQKPGKAPKLLIYAASSLQSGVPSRFSGSGSGTDFTLTISSLQPEDFATYYCQQSYSTPPTFGQGTKVEIKRAAAGSTSGSGKPGSGEGSTKGAEVQLVESGGGLVQPGGSLRLPCAASGFTFSNYVMHWVRQAPGKGLEWVAVISYDGSNKYYADSVKGRFTISRDNSKNTLYLQMNSLRAEDTAVYYCAKSHSNMSFDYWGQGTLVTVESKYGPPCPPCPMFWVLVVVGGVLACYSLLVTVAFIIFWVKRGRKKLLYIFKQPFMRPVQTTQEEDGCSCRFPEEEEGGCELRVKFSRSADAPAYQQGQNQLYNELNLGRREEYDVLDKRRGRDPEMGGKPRRKNPQEGLYNELQKDKMAEAYSEIGMKGERRRGKGHDGLYQGLSTATKDTYDALHMQALPPR

SEQ ID NO: 206 - protein, 439 aa, synthetic construct
AEVQLVESGGGLVQPGGSLRLPCAASGFTFSNYVMHWVRQAPGKGLEWVAVISYDGSNKYYADSVKGRFTISRDNSKNTLYLQMNSLRAEDTAVYYCAKSHSNMSFDYWGQGTLVTVGSTSGSGKPGSGEGSTKGSELTQSPSSLSASVGDRVTITCRASQSISSYLNWYQQKPGKAPKLLIYAASSLQSGVPSRFSGSGSGTDFTLTISSLQPEDFATYYCQQSYSTPPTFGQGTKVEIKRAAAESKYGPPCPPCPMFWVLVVVGGVLACYSLLVTVAFIIFWVKRGRKKLLYIFKQPFMRPVQTTQEEDGCSCRFPEEEEGGCELRVKFSRSADAPAYQQGQNQLYNELNLGRREEYDVLDKRRGRDPEMGGKPRRKNPQEGLYNELQKDKMAEAYSEIGMKGERRRGKGHDGLYQGLSTATKDTYDALHMQALPPR

SEQ ID NO: 207 - protein, 440 aa, synthetic construct
SELTQSPSSLSASVGDRVTITCRASQSISSYLNWYQQKPGKAPKLLIYAASSLQSGVPSRFSGSGSGTDFTLTISSLQPEDFATYYCQQSYSTPPTFGQGTKVEIKRAAAGSTSGSGKPGSGEGSTKGAEVQLVESGGGLVQPGGSLRLSCAASGFTFSGYLMSWVRQAPGKGLEWVAVISYDGSNKYYADSVKGRFTISRDNSKNTLYLQMDSLRAEDTAVYYCARARRDTNLFDYWGQGTLVTVESKYGPPCPPCPMFWVLVVVGGVLACYSLLVTVAFIIFWVKRGRKKLLYIFKQPFMRPVQTTQEEDGCSCRFPEEEEGGCELRVKFSRSADAPAYQQGQNQLYNELNLGRREEYDVLDKRRGRDPEMGGKPRRKNPQEGLYNELQKDKMAEAYSEIGMKGERRRGKGHDGLYQGLSTATKDTYDALHMQALPPR

SEQ ID NO: 208 - protein, 440 aa, synthetic construct
AEVQLVESGGGLVQPGGSLRLSCAASGFTFSGYLMSWVRQAPGKGLEWVAVISYDGSNKYYADSVKGRFTISRDNSKNTLYLQMDSLRAEDTAVYYCARARRDTNLFDYWGQGTLVTVGSTSGSGKPGSGEGSTKGSELTQSPSSLSASVGDRVTITCRASQSISSYLNWYQQKPGKAPKLLIYAASSLQSGVPSRFSGSGSGTDFTLTISSLQPEDFATYYCQQSYSTPPTFGQGTKVEIKRAAAESKYGPPCPPCPMFWVLVVVGGVLACYSLLVTVAFIIFWVKRGRKKLLYIFKQPFMRPVQTTQEEDGCSCRFPEEEEGGCELRVKFSRSADAPAYQQGQNQLYNELNLGRREEYDVLDKRRGRDPEMGGKPRRKNPQEGLYNELQKDKMAEAYSEIGMKGERRRGKGHDGLYQGLSTATKDTYDALHMQALPPR

SEQ ID NO: 209 - protein, 444 aa, synthetic construct
SEIELTQSPSSLSASVGDRVTITCRASQSISSYLNWYQQKPGKAPKLLIYAASSLQSGVPSRFSGSGSGTDFTLTISSLQPEDFATYYCQQSYSTPPTFGQGTKVEIKRAAAGSTSGSGKPGSGEGSTKGAQVQLVQSGPEVKKPGASVKVSCKASGYTFTSYYMHWVRQAPGQGLEWMGIINPSGGSTSYAQKFQGRVTMTRDTSTSTVYMELSSLRSEDAAVYYCARDYVRTSHSGFDYWGQGTLVTVESKYGPPCPPCPMFWVLVVVGGVLACYSLLVTVAFIIFWVKRGRKKLLYIFKQPFMRPVQTTQEEDGCSCRFPEEEEGGCELRVKFSRSADAPAYQQGQNQLYNELNLGRREEYDVLDKRRGRDPEMGGKPRRKNPQEGLYNELQKDKMAEAYSEIGMKGERRRGKGHDGLYQGLSTATKDTYDALHMQALPPR

SEQ ID NO: 210 - protein, 444 aa, synthetic construct
AQVQLVQSGPEVKKPGASVKVSCKASGYTFTSYYMHWVRQAPGQGLEWMGIINPSGGSTSYAQKFQGRVTMTRDTSTSTVYMELSSLRSEDAAVYYCARDYVRTSHSGFDYWGQGTLVTVGSTSGSGKPGSGEGSTKGSEIELTQSPSSLSASVGDRVTITCRASQSISSYLNWYQQKPGKAPKLLIYAASSLQSGVPSRFSGSGSGTDFTLTISSLQPEDFATYYCQQSYSTPPTFGQGTKVEIKRAAAESKYGPPCPPCPMFWVLVVVGGVLACYSLLVTVAFIIFWVKRGRKKLLYIFKQPFMRPVQTTQEEDGCSCRFPEEEEGGCELRVKFSRSADAPAYQQGQNQLYNELNLGRREEYDVLDKRRGRDPEMGGKPRRKNPQEGLYNELQKDKMAEAYSEIGMKGERRRGKGHDGLYQGLSTATKDTYDALHMQALPPR

SEQ ID NO: 211 - protein, 444 aa, synthetic construct
SELTQDPAVSVALGQTVRITCQGDSLRSYYASWYQQKPGQAPVLVIYGKNNRPSGIPDRFSGSSSGNTASLTITGAQAEDEADYYCNSRDSSGNHVVFGGGTKLTVLGAAAGSTSGSGKPGSGEGSTKGAQVQLVQSGAEVKKPGASVKVSCKASGYTFTSYYMHWVRQAPGQGLEWMGIINPSGGGTSYAQKFQGRVTMTRDTSTSTVYMELSSLRSEDTAVYYCARDYYVTYDSWFDSWGQGTLVTVSESKYGPPCPPCPMFWVLVVVGGVLACYSLLVTVAFIIFWVKRGRKKLLYIFKQPFMRPVQTTQEEDGCSCRFPEEEEGGCELRVKFSRSADAPAYQQGQNQLYNELNLGRREEYDVLDKRRGRDPEMGGKPRRKNPQEGLYNELQKDKMAEAYSEIGMKGERRRGKGHDGLYQGLSTATKDTYDALHMQALPPR

SEQ ID NO: 212 - protein, 444 aa, synthetic construct
AQVQLVQSGAEVKKPGASVKVSCKASGYTFTSYYMHWVRQAPGQGLEWMGIINPSGGGTSYAQKFQGRVTMTRDTSTSTVYMELSSLRSEDTAVYYCARDYYVTYDSWFDSWGQGTLVTVSGSTSGSGKPGSGEGSTKGSELTQDPAVSVALGQTVRITCQGDSLRSYYASWYQQKPGQAPVLVIYGKNNRPSGIPDRFSGSSSGNTASLTITGAQAEDEADYYCNSRDSSGNHVVFGGGTKLTVLGAAAESKYGPPCPPCPMFWVLVVVGGVLACYSLLVTVAFIIFWVKRGRKKLLYIFKQPFMRPVQTTQEEDGCSCRFPEEEEGGCELRVKFSRSADAPAYQQGQNQLYNELNLGRREEYDVLDKRRGRDPEMGGKPRRKNPQEGLYNELQKDKMAEAYSEIGMKGERRRGKGHDGLYQGLSTATKDTYDALHMQALPPR

SEQ ID NO: 213 - protein, 439 aa, synthetic construct
SELTQSPSSLSASVGDRVTITCRASQSISSYLNWYQQKPGKAPKLLIYAASSLQSGVPSRFSGSGSGTDFTLTISSLQPEDFATYYCQQSYSTPPTFGQGTKVEIKRAAAGSTSGSGKPGSGEGSTKGAEVQLVESGGGLVQPGGSLRLPCAASGFTFSNYVMHWVRQAPGKGLEWVAVISYDGSNKYYADSVKGRFTISRDNSKNTLYLQMNSLRAEDTAVYYCAKSHSNMAFDYWGQGTLVTVESKYGPPCPPCPMFWVLVVVGGVLACYSLLVTVAFIIFWVKRGRKKLLYIFKQPFMRPVQTTQEEDGCSCRFPEEEEGGCELRVKFSRSADAPAYQQGQNQLYNELNLGRREEYDVLDKRRGRDPEMGGKPRRKNPQEGLYNELQKDKMAEAYSEIGMKGERRRGKGHDGLYQGLSTATKDTYDALHMQALPPR

SEQ ID NO: 214 - protein, 439 aa, synthetic construct
AEVQLVESGGGLVQPGGSLRLPCAASGFTFSNYVMHWVRQAPGKGLEWVAVISYDGSNKYYADSVKGRFTISRDNSKNTLYLQMNSLRAEDTAVYYCAKSHSNMAFDYWGQGTLVTVGSTSGSGKPGSGEGSTKGSELTQSPSSLSASVGDRVTITCRASQSISSYLNWYQQKPGKAPKLLIYAASSLQSGVPSRFSGSGSGTDFTLTISSLQPEDFATYYCQQSYSTPPTFGQGTKVEIKRAAAESKYGPPCPPCPMFWVLVVVGGVLACYSLLVTVAFIIFWVKRGRKKLLYIFKQPFMRPVQTTQEEDGCSCRFPEEEEGGCELRVKFSRSADAPAYQQGQNQLYNELNLGRREEYDVLDKRRGRDPEMGGKPRRKNPQEGLYNELQKDKMAEAYSEIGMKGERRRGKGHDGLYQGLSTATKDTYDALHMQALPPR

SEQ ID NO: 215 - protein, 444 aa, synthetic construct
SEIELTQSPSSLSASVGDRVTITCRASQSISSYLNWYQQKPGKAPKLLIYAASSLQSGVPSRFSGSGSGTDFTLTISSLQPEDFATYYCQQSYSTPPTFGQGTKVEIKRAAAGSTSGSGKPGSGEGSTKGAQVQLVQSGAEVKKPGASVKVSCKASGYTFTSYYMHWVRQAPGQGLEWMGIINPSGGSTSYAQKFQGRVTMTRDTSTSTVYMELSSLRSEDTAVYYCARDYQLSMTSGFDYWGQGTLVTVESKYGPPCPPCPMFWVLVVVGGVLACYSLLVTVAFIIFWVKRGRKKLLYIFKQPFMRPVQTTQEEDGCSCRFPEEEEGGCELRVKFSRSADAPAYQQGQNQLYNELNLGRREEYDVLDKRRGRDPEMGGKPRRKNPQEGLYNELQKDKMAEAYSEIGMKGERRRGKGHDGLYQGLSTATKDTYDALHMQALPPR

SEQ ID NO: 216 - protein, 444 aa, synthetic construct
AQVQLVQSGAEVKKPGASVKVSCKASGYTFTSYYMHWVRQAPGQGLEWMGIINPSGGSTSYAQKFQGRVTMTRDTSTSTVYMELSSLRSEDTAVYYCARDYQLSMTSGFDYWGQGTLVTVGSTSGSGKPGSGEGSTKGSEIELTQSPSSLSASVGDRVTITCRASQSISSYLNWYQQKPGKAPKLLIYAASSLQSGVPSRFSGSGSGTDFTLTISSLQPEDFATYYCQQSYSTPPTFGQGTKVEIKRAAAESKYGPPCPPCPMFWVLVVVGGVLACYSLLVTVAFIIFWVKRGRKKLLYIFKQPFMRPVQTTQEEDGCSCRFPEEEEGGCELRVKFSRSADAPAYQQGQNQLYNELNLGRREEYDVLDKRRGRDPEMGGKPRRKNPQEGLYNELQKDKMAEAYSEIGMKGERRRGKGHDGLYQGLSTATKDTYDALHMQALPPR

SEQ ID NO: 217 - protein, 439 aa, synthetic construct
SELTQSPSSLSASVGDRVTITCRASQSISSYLNWYQQKPGKAPKLLIYAASSLQSGVPSRFSGSGSGTDFTLTISSLQPEDFATYYCQQSYSTPPTFGQGTKVEIKRAAAGSTSGSGKPGSGEGSTKGAEVQLVESGGGLVQPGGSLRLPCAASGFTFSNYVMHWVRQAPGKGLEWVAVISYDGSNKYYADSVKGRFTISRDNSKNTLYLQMNSLRAEDTAVYYCVKSHSNMAFDYWGQGTLVTVESKYGPPCPPCPMFWVLVVVGGVLACYSLLVTVAFIIFWVKRGRKKLLYIFKQPFMRPVQTTQEEDGCSCRFPEEEEGGCELRVKFSRSADAPAYQQGQNQLYNELNLGRREEYDVLDKRRGRDPEMGGKPRRKNPQEGLYNELQKDKMAEAYSEIGMKGERRRGKGHDGLYQGLSTATKDTYDALHMQALPPR

SEQ ID NO: 218 - protein, 439 aa, synthetic construct
AEVQLVESGGGLVQPGGSLRLPCAASGFTFSNYVMHWVRQAPGKGLEWVAVISYDGSNKYYADSVKGRFTISRDNSKNTLYLQMNSLRAEDTAVYYCVKSHSNMAFDYWGQGTLVTVGSTSGSGKPGSGEGSTKGSELTQSPSSLSASVGDRVTITCRASQSISSYLNWYQQKPGKAPKLLIYAASSLQSGVPSRFSGSGSGTDFTLTISSLQPEDFATYYCQQSYSTPPTFGQGTKVEIKRAAAESKYGPPCPPCPMFWVLVVVGGVLACYSLLVTVAFIIFWVKRGRKKLLYIFKQPFMRPVQTTQEEDGCSCRFPEEEEGGCELRVKFSRSADAPAYQQGQNQLYNELNLGRREEYDVLDKRRGRDPEMGGKPRRKNPQEGLYNELQKDKMAEAYSEIGMKGERRRGKGHDGLYQGLSTATKDTYDALHMQALPPR

SEQ ID NO: 219 - protein, 445 aa, synthetic construct
SELDIQMTQSPPTLSLSPGERATLSCRASQSVSSTYLTWYQQRPGQAPRLLIYGASSRATGIPDRFSGSGSGTDFTLTISRLEPEDVAVYYCQQGSAFPPTFGQGTKVEIKRAAALEGTGGSGGTGSGTGTAEVQLVESGGGVVQPGRSLRLSCAASGFTFSDYTMSWVRQAPGKGLEWVAVISYDGSNKYYADSVKGRFTISRDNSKNTLYLQMNSLRAEDTAVYYCAKDRGSAQGYPLDYWGQGTLVTVESKYGPPCPPCPMFWVLVVVGGVLACYSLLVTVAFIIFWVKRGRKKLLYIFKQPFMRPVQTTQEEDGCSCRFPEEEEGGCELRVKFSRSADAPAYQQGQNQLYNELNLGRREEYDVLDKRRGRDPEMGGKPRRKNPQEGLYNELQKDKMAEAYSEIGMKGERRRGKGHDGLYQGLSTATKDTYDALHMQALPPR

SEQ ID NO: 220 - protein, 445 aa, synthetic construct
AEVQLVESGGGVVQPGRSLRLSCAASGFTFSDYTMSWVRQAPGKGLEWVAVISYDGSNKYYADSVKGRFTISRDNSKNTLYLQMNSLRAEDTAVYYCAKDRGSAQGYPLDYWGQGTLVTVLEGTGGSGGTGSGTGTSELDIQMTQSPPTLSLSPGERATLSCRASQSVSSTYLTWYQQRPGQAPRLLIYGASSRATGIPDRFSGSGSGTDFTLTISRLEPEDVAVYYCQQGSAFPPTFGQGTKVEIKRAAAESKYGPPCPPCPMFWVLVVVGGVLACYSLLVTVAFIIFWVKRGRKKLLYIFKQPFMRPVQTTQEEDGCSCRFPEEEEGGCELRVKFSRSADAPAYQQGQNQLYNELNLGRREEYDVLDKRRGRDPEMGGKPRRKNPQEGLYNELQKDKMAEAYSEIGMKGERRRGKGHDGLYQGLSTATKDTYDALHMQALPPR

SEQ ID NO: 221 - protein, 437 aa, synthetic construct
SELTQSPSSLSASVGDRVTITCRASQSISSYLNWYQQKPGKAPKLLIYAASSLQSGVPSRFSGSGSGTDFTLTISSLQPEDFATYYCQQSYSTPPTFGQGTKVEIKRAAALEGTGGSGGTGSGTGTAEVQLVESGGGLVQPGGSLRLPCAASGFTFSNYVMHWVRQAPGKGLEWVAVISYDGSNKYYADSVKGRFTISRDNSKNTLYLQMNSLRAEDTAVYYCAKSHSNMSFDYWGQGTLVTVESKYGPPCPPCPMFWVLVVVGGVLACYSLLVTVAFIIFWVKRGRKKLLYIFKQPFMRPVQTTQEEDGCSCRFPEEEEGGCELRVKFSRSADAPAYQQGQNQLYNELNLGRREEYDVLDKRRGRDPEMGGKPRRKNPQEGLYNELQKDKMAEAYSEIGMKGERRRGKGHDGLYQGLSTATKDTYDALHMQALPPR

SEQ ID NO: 222 - protein, 437 aa, synthetic construct
AEVQLVESGGGLVQPGGSLRLPCAASGFTFSNYVMHWVRQAPGKGLEWVAVISYDGSNKYYADSVKGRFTISRDNSKNTLYLQMNSLRAEDTAVYYCAKSHSNMSFDYWGQGTLVTVLEGTGGSGGTGSGTGTSELTQSPSSLSASVGDRVTITCRASQSISSYLNWYQQKPGKAPKLLIYAASSLQSGVPSRFSGSGSGTDFTLTISSLQPEDFATYYCQQSYSTPPTFGQGTKVEIKRAAAESKYGPPCPPCPMFWVLVVVGGVLACYSLLVTVAFIIFWVKRGRKKLLYIFKQPFMRPVQTTQEEDGCSCRFPEEEEGGCELRVKFSRSADAPAYQQGQNQLYNELNLGRREEYDVLDKRRGRDPEMGGKPRRKNPQEGLYNELQKDKMAEAYSEIGMKGERRRGKGHDGLYQGLSTATKDTYDALHMQALPPR

SEQ ID NO: 223 - protein, 438 aa, synthetic construct
SELTQSPSSLSASVGDRVTITCRASQSISSYLNWYQQKPGKAPKLLIYAASSLQSGVPSRFSGSGSGTDFTLTISSLQPEDFATYYCQQSYSTPPTFGQGTKVEIKRAAALEGTGGSGGTGSGTGTAEVQLVESGGGLVQPGGSLRLSCAASGFTFSGYLMSWVRQAPGKGLEWVAVISYDGSNKYYADSVKGRFTISRDNSKNTLYLQMDSLRAEDTAVYYCARARRDTNLFDYWGQGTLVTVESKYGPPCPPCPMFWVLVVVGGVLACYSLLVTVAFIIFWVKRGRKKLLYIFKQPFMRPVQTTQEEDGCSCRFPEEEEGGCELRVKFSRSADAPAYQQGQNQLYNELNLGRREEYDVLDKRRGRDPEMGGKPRRKNPQEGLYNELQKDKMAEAYSEIGMKGERRRGKGHDGLYQGLSTATKDTYDALHMQALPPR

SEQ ID NO: 224 - protein, 438 aa, synthetic construct
AEVQLVESGGGLVQPGGSLRLSCAASGFTFSGYLMSWVRQAPGKGLEWVAVISYDGSNKYYADSVKGRFTISRDNSKNTLYLQMDSLRAEDTAVYYCARARRDTNLFDYWGQGTLVTVLEGTGGSGGTGSGTGTSELTQSPSSLSASVGDRVTITCRASQSISSYLNWYQQKPGKAPKLLIYAASSLQSGVPSRFSGSGSGTDFTLTISSLQPEDFATYYCQQSYSTPPTFGQGTKVEIKRAAAESKYGPPCPPCPMFWVLVVVGGVLACYSLLVTVAFIIFWVKRGRKKLLYIFKQPFMRPVQTTQEEDGCSCRFPEEEEGGCELRVKFSRSADAPAYQQGQNQLYNELNLGRREEYDVLDKRRGRDPEMGGKPRRKNPQEGLYNELQKDKMAEAYSEIGMKGERRRGKGHDGLYQGLSTATKDTYDALHMQALPPR

SEQ ID NO: 225 - protein, 442 aa, synthetic construct
SEIELTQSPSSLSASVGDRVTITCRASQSISSYLNWYQQKPGKAPKLLIYAASSLQSGVPSRFSGSGSGTDFTLTISSLQPEDFATYYCQQSYSTPPTFGQGTKVEIKRAAASSGGGGSGGGGSGGGGAQVQLVQSGPEVKKPGASVKVSCKASGYTFTSYYMHWVRQAPGQGLEWMGIINPSGGSTSYAQKFQGRVTMTRDTSTSTVYMELSSLRSEDAAVYYCARDYVRTSHSGFDYWGQGTLVTVESKYGPPCPPCPMFWVLVVVGGVLACYSLLVTVAFIIFWVKRGRKKLLYIFKQPFMRPVQTTQEEDGCSCRFPEEEEGGCELRVKFSRSADAPAYQQGQNQLYNELNLGRREEYDVLDKRRGRDPEMGGKPRRKNPQEGLYNELQKDKMAEAYSEIGMKGERRRGKGHDGLYQGLSTATKDTYDALHMQALPPR

SEQ ID NO: 226 - protein, 442 aa, synthetic construct
AQVQLVQSGPEVKKPGASVKVSCKASGYTFTSYYMHWVRQAPGQGLEWMGIINPSGGSTSYAQKFQGRVTMTRDTSTSTVYMELSSLRSEDAAVYYCARDYVRTSHSGFDYWGQGTLVTVSSGGGGSGGGGSGGGGSEIELTQSPSSLSASVGDRVTITCRASQSISSYLNWYQQKPGKAPKLLIYAASSLQSGVPSRFSGSGSGTDFTLTISSLQPEDFATYYCQQSYSTPPTFGQGTKVEIKRAAAESKYGPPCPPCPMFWVLVVVGGVLACYSLLVTVAFIIFWVKRGRKKLLYIFKQPFMRPVQTTQEEDGCSCRFPEEEEGGCELRVKFSRSADAPAYQQGQNQLYNELNLGRREEYDVLDKRRGRDPEMGGKPRRKNPQEGLYNELQKDKMAEAYSEIGMKGERRRGKGHDGLYQGLSTATKDTYDALHMQALPPR

SEQ ID NO: 227 - protein, 442 aa, synthetic construct
SELTQDPAVSVALGQTVRITCQGDSLRSYYASWYQQKPGQAPVLVIYGKNNRPSGIPDRFSGSSSGNTASLTITGAQAEDEADYYCNSRDSSGNHVVFGGGTKLTVLGAAARGGGGSGGGGSGGGGSAQVQLVQSGAEVKKPGASVKVSCKASGYTFTSYYMHWVRQAPGQGLEWMGIINPSGGGTSYAQKFQGRVTMTRDTSTSTVYMELSSLRSEDTAVYYCARDYYVTYDSWFDSWGQGTLVTVSESKYGPPCPPCPMFWVLVVVGGVLACYSLLVTVAFIIFWVKRGRKKLLYIFKQPFMRPVQTTQEEDGCSCRFPEEEEGGCELRVKFSRSADAPAYQQGQNQLYNELNLGRREEYDVLDKRRGRDPEMGGKPRRKNPQEGLYNELQKDKMAEAYSEIGMKGERRRGKGHDGLYQGLSTATKDTYDALHMQALPPR

SEQ ID NO: 228 - protein, 442 aa, synthetic construct
AQVQLVQSGAEVKKPGASVKVSCKASGYTFTSYYMHWVRQAPGQGLEWMGIINPSGGGTSYAQKFQGRVTMTRDTSTSTVYMELSSLRSEDTAVYYCARDYYVTYDSWFDSWGQGTLVTVSRGGGGSGGGGSGGGGSSELTQDPAVSVALGQTVRITCQGDSLRSYYASWYQQKPGQAPVLVIYGKNNRPSGIPDRFSGSSSGNTASLTITGAQAEDEADYYCNSRDSSGNHVVFGGGTKLTVLGAAAESKYGPPCPPCPMFWVLVVVGGVLACYSLLVTVAFIIFWVKRGRKKLLYIFKQPFMRPVQTTQEEDGCSCRFPEEEEGGCELRVKFSRSADAPAYQQGQNQLYNELNLGRREEYDVLDKRRGRDPEMGGKPRRKNPQEGLYNELQKDKMAEAYSEIGMKGERRRGKGHDGLYQGLSTATKDTYDALHMQALPPR

SEQ ID NO: 229 - protein, 437 aa, synthetic construct
SELTQSPSSLSASVGDRVTITCRASQSISSYLNWYQQKPGKAPKLLIYAASSLQSGVPSRFSGSGSGTDFTLTISSLQPEDFATYYCQQSYSTPPTFGQGTKVEIKRAAALEGTGGSGGTGSGTGTAEVQLVESGGGLVQPGGSLRLPCAASGFTFSNYVMHWVRQAPGKGLEWVAVISYDGSNKYYADSVKGRFTISRDNSKNTLYLQMNSLRAEDTAVYYCAKSHSNMAFDYWGQGTLVTVESKYGPPCPPCPMFWVLVVVGGVLACYSLLVTVAFIIFWVKRGRKKLLYIFKQPFMRPVQTTQEEDGCSCRFPEEEEGGCELRVKFSRSADAPAYQQGQNQLYNELNLGRREEYDVLDKRRGRDPEMGGKPRRKNPQEGLYNELQKDKMAEAYSEIGMKGERRRGKGHDGLYQGLSTATKDTYDALHMQALPPR

SEQ ID NO: 230 - protein, 437 aa, synthetic construct
AEVQLVESGGGLVQPGGSLRLPCAASGFTFSNYVMHWVRQAPGKGLEWVAVISYDGSNKYYADSVKGRFTISRDNSKNTLYLQMNSLRAEDTAVYYCAKSHSNMAFDYWGQGTLVTVLEGTGGSGGTGSGTGTSELTQSPSSLSASVGDRVTITCRASQSISSYLNWYQQKPGKAPKLLIYAASSLQSGVPSRFSGSGSGTDFTLTISSLQPEDFATYYCQQSYSTPPTFGQGTKVEIKRAAAESKYGPPCPPCPMFWVLVVVGGVLACYSLLVTVAFIIFWVKRGRKKLLYIFKQPFMRPVQTTQEEDGCSCRFPEEEEGGCELRVKFSRSADAPAYQQGQNQLYNELNLGRREEYDVLDKRRGRDPEMGGKPRRKNPQEGLYNELQKDKMAEAYSEIGMKGERRRGKGHDGLYQGLSTATKDTYDALHMQALPPR

SEQ ID NO: 231 - protein, 442 aa, synthetic construct
SEIELTQSPSSLSASVGDRVTITCRASQSISSYLNWYQQKPGKAPKLLIYAASSLQSGVPSRFSGSGSGTDFTLTISSLQPEDFATYYCQQSYSTPPTFGQGTKVEIKRAAASSGGGGSGGGGSGGGGAQVQLVQSGAEVKKPGASVKVSCKASGYTFTSYYMHWVRQAPGQGLEWMGIINPSGGSTSYAQKFQGRVTMTRDTSTSTVYMELSSLRSEDTAVYYCARDYQLSMTSGFDYWGQGTLVTVESKYGPPCPPCPMFWVLVVVGGVLACYSLLVTVAFIIFWVKRGRKKLLYIFKQPFMRPVQTTQEEDGCSCRFPEEEEGGCELRVKFSRSADAPAYQQGQNQLYNELNLGRREEYDVLDKRRGRDPEMGGKPRRKNPQEGLYNELQKDKMAEAYSEIGMKGERRRGKGHDGLYQGLSTATKDTYDALHMQALPPR

SEQ ID NO: 232 - protein, 442 aa, synthetic construct
AQVQLVQSGAEVKKPGASVKVSCKASGYTFTSYYMHWVRQAPGQGLEWMGIINPSGGSTSYAQKFQGRVTMTRDTSTSTVYMELSSLRSEDTAVYYCARDYQLSMTSGFDYWGQGTLVTVSSGGGGSGGGGSGGGGSEIELTQSPSSLSASVGDRVTITCRASQSISSYLNWYQQKPGKAPKLLIYAASSLQSGVPSRFSGSGSGTDFTLTISSLQPEDFATYYCQQSYSTPPTFGQGTKVEIKRAAAESKYGPPCPPCPMFWVLVVVGGVLACYSLLVTVAFIIFWVKRGRKKLLYIFKQPFMRPVQTTQEEDGCSCRFPEEEEGGCELRVKFSRSADAPAYQQGQNQLYNELNLGRREEYDVLDKRRGRDPEMGGKPRRKNPQEGLYNELQKDKMAEAYSEIGMKGERRRGKGHDGLYQGLSTATKDTYDALHMQALPPR

SEQ ID NO: 233 - protein, 437 aa, synthetic construct
SELTQSPSSLSASVGDRVTITCRASQSISSYLNWYQQKPGKAPKLLIYAASSLQSGVPSRFSGSGSGTDFTLTISSLQPEDFATYYCQQSYSTPPTFGQGTKVEIKRAAALEGTGGSGGTGSGTGTAEVQLVESGGGLVQPGGSLRLPCAASGFTFSNYVMHWVRQAPGKGLEWVAVISYDGSNKYYADSVKGRFTISRDNSKNTLYLQMNSLRAEDTAVYYCVKSHSNMAFDYWGQGTLVTVESKYGPPCPPCPMFWVLVVVGGVLACYSLLVTVAFIIFWVKRGRKKLLYIFKQPFMRPVQTTQEEDGCSCRFPEEEEGGCELRVKFSRSADAPAYQQGQNQLYNELNLGRREEYDVLDKRRGRDPEMGGKPRRKNPQEGLYNELQKDKMAEAYSEIGMKGERRRGKGHDGLYQGLSTATKDTYDALHMQALPPR

SEQ ID NO: 234 - protein, 437 aa, synthetic construct
AEVQLVESGGGLVQPGGSLRLPCAASGFTFSNYVMHWVRQAPGKGLEWVAVISYDGSNKYYADSVKGRFTISRDNSKNTLYLQMNSLRAEDTAVYYCVKSHSNMAFDYWGQGTLVTVLEGTGGSGGTGSGTGTSELTQSPSSLSASVGDRVTITCRASQSISSYLNWYQQKPGKAPKLLIYAASSLQSGVPSRFSGSGSGTDFTLTISSLQPEDFATYYCQQSYSTPPTFGQGTKVEIKRAAAESKYGPPCPPCPMFWVLVVVGGVLACYSLLVTVAFIIFWVKRGRKKLLYIFKQPFMRPVQTTQEEDGCSCRFPEEEEGGCELRVKFSRSADAPAYQQGQNQLYNELNLGRREEYDVLDKRRGRDPEMGGKPRRKNPQEGLYNELQKDKMAEAYSEIGMKGERRRGKGHDGLYQGLSTATKDTYDALHMQALPPR

SEQ ID NO: 235 - protein, 21 aa, Homo sapiens
MLLVTSLLLCELPHPAFLLIP

SEQ ID NO: 236 - protein, 20 aa, Homo sapiens
MVLQTQVFISLLLWISGAYG

SEQ ID NO: 237 - protein, 18 aa, Homo sapiens
MALPVTALLLPLALLLHA

SEQ ID NO: 238 - protein, 20 aa, Homo sapiens
MYRMQLLSCIALSLALVTNS

SEQ ID NO: 239 - protein, 10 aa, synthetic construct
EQKLISEEDL

SEQ ID NO: 240 - protein, 22 aa, Homo sapiens
MLLLVTSLLLCELPHPAFLLIP

SEQ ID NO: 241 - protein, 598 aa, synthetic construct
MAPGLLCWALLCLLGAGLVDAGVTQSPTHLIKTRGQQVTLRCSPKSGHDTVSWYQQALGQGPQFIFQYYEEEERQRGNFPDRFSGHQFPNYSSELNVNALLLGDSALYLCASSLGWRGGRYNEQFFGPGTRLTVLEDLRNVTPPKVSLFEPSKAEIANKQKATLVCLARGFFPDHVELSWWVNGKEVHSGVCTDPQAYKESNYSYCLSSRLRVSATFWHNPRNHFRCQVQFHGLSEEDKWPEGSPKPVTQNISAEAWGRADCGITSASYQQGVLSATILYEILLGKATLYAVLVSTLVVMAMVKRKNSRAKRSGSGATNFSLLKQAGDVEENPGPMWGVFLLYVSMKMGGTTGQNIDQPTEMTATEGAIVQINCTYQTSGFNGLFWYQQHAGEAPTFLSYNVLDGLEEKGRFSSFLSRSKGYSYLLLKELQMKDSASYLCASVDGNNRLAFGKGNQVVVIPNIQNPEPAVYQLKDPRSQDSTLCLFTDFDSQINVPKTMESGTFITDKCVLDMKAMDSKSNGAIAWSNQTSFTCQDIFKETNATYPSSDVPCDATLTEKSFETDMNLNFQNLLVIVLRILLLKVAGFNLLMTLRLWSS

SEQ ID NO: 242-301 - skipped (60 entries)

SEQ ID NO: 302 - protein, 6 aa, synthetic construct
GFTFSD

SEQ ID NO: 303 - protein, 8 aa, synthetic construct
ISYDGSNK

SEQ ID NO: 304 - protein, 14 aa, synthetic construct
AKDRGSAQGYPLDY

SEQ ID NO: 305 - protein, 7 aa, synthetic construct
QSVSSTY

SEQ ID NO: 306 - skipped

SEQ ID NO: 307 - protein, 7 aa, synthetic construct
QQGSAFP

SEQ ID NO: 308 - protein, 8 aa, synthetic construct
GFTFSNYV

SEQ ID NO: 309 - protein, 8 aa, synthetic construct
ISYDGSNK

SEQ ID NO: 310 - protein, 11 aa, synthetic construct
AKSHSNMSFDY

SEQ ID NO: 311 - protein, 6 aa, synthetic construct
FTEHFQ

SEQ ID NO: 312 - skipped

SEQ ID NO: 313 - protein, 7 aa, synthetic construct
QQSYSTP

SEQ ID NO: 314 - protein, 8 aa, synthetic construct
GFTFSGYL

SEQ ID NO: 315 - protein, 8 aa, synthetic construct
ISYDGSNK

SEQ ID NO: 316 - protein, 12 aa, synthetic construct
ARARRDTNLFDY

SEQ ID NO: 317 - protein, 6 aa, synthetic construct
QSISSY

SEQ ID NO: 318 - skipped

SEQ ID NO: 319 - protein, 9 aa, synthetic construct
QQSYSTPPT

SEQ ID NO: 320 - protein, 8 aa, synthetic construct
GYTFTSYY

SEQ ID NO: 321 - protein, 8 aa, synthetic construct
INPSGGST

SEQ ID NO: 322 - protein, 13 aa, synthetic construct
ARDYVRTSHSGFD

SEQ ID NO: 323 - protein, 6 aa, synthetic construct
QSISSY

SEQ ID NO: 324 - skipped

SEQ ID NO: 325 - protein, 9 aa, synthetic construct
QQSYSTPPT

SEQ ID NO: 326 - protein, 8 aa, synthetic construct
GYTFTSYY

SEQ ID NO: 327 - protein, 8 aa, synthetic construct
INPSGGGT

SEQ ID NO: 328 - protein, 14 aa, synthetic construct
ARDYYVTYDSWFDS

SEQ ID NO: 329 - protein, 6 aa, synthetic construct
SLRSYY

SEQ ID NO: 330 - skipped

SEQ ID NO: 331 - protein, 11 aa, synthetic construct
NSRDSSGNHVV

SEQ ID NO: 332 - protein, 8 aa, synthetic construct
GFTFSNYV

SEQ ID NO: 333 - protein, 8 aa, synthetic construct
ISYDGSNK

SEQ ID NO: 334 - protein, 11 aa, synthetic construct
AKSHSNMAFDY

SEQ ID NO: 335 - protein, 6 aa, synthetic construct
QSISSY

SEQ ID NO: 336 - skipped

SEQ ID NO: 337 - protein, 9 aa, synthetic construct
QQSYSTPPT

SEQ ID NO: 338 - protein, 8 aa, synthetic construct
GYTFTSYY

SEQ ID NO: 339 - protein, 8 aa, synthetic construct
INPSGGST

SEQ ID NO: 340 - protein, 14 aa, synthetic construct
ARDYQLSMTSGFDY

SEQ ID NO: 341 - protein, 6 aa, synthetic construct
QSISSY

SEQ ID NO: 342 - skipped

SEQ ID NO: 343 - protein, 9 aa, synthetic construct
QQSYSTPPT

SEQ ID NO: 344 - protein, 8 aa, synthetic construct
GFTFSNYV

SEQ ID NO: 345 - protein, 8 aa, synthetic construct
ISYDGSNK

SEQ ID NO: 346 - protein, 11 aa, synthetic construct
VKSHSNMAFDY

SEQ ID NO: 347 - protein, 6 aa, synthetic construct
QSISSY

SEQ ID NO: 348 - skipped

SEQ ID NO: 349 - protein, 9 aa, synthetic construct
QQSYSTPPT